European Patent Application EP 4 741 502 A1, published May 13, 2026. Title: 一种抑制LP(a)基因表达的dsRNA分子及其应用. Applicant: 石药集团中奇制药技术（石家庄）有限公司. The sequence listing filed with the application follows.

SEQUENCE LISTING (796 sequences)

SEQ ID NO: 1 - RNA, 21 nt, synthetic construct
  source 1..21: mol_type = other RNA
  modified_base 1..21: mod_base = OTHER; note = modified as descibed in table 8
agagttatcgaggcacgtact

SEQ ID NO: 2 - RNA, 23 nt, synthetic construct
  source 1..23: mol_type = other RNA
  modified_base 1..23: mod_base = OTHER; note = modified as descibed in table 8
agtacgtgcctcgataactctgt

SEQ ID NO: 3 - RNA, 21 nt, synthetic construct
  source 1..21: mol_type = other RNA
  modified_base 1..21: mod_base = OTHER; note = modified as descibed in table 8
gaggcacgtactccaccactg

SEQ ID NO: 4 - RNA, 23 nt, synthetic construct
  source 1..23: mol_type = other RNA
  modified_base 1..23: mod_base = OTHER; note = modified as descibed in table 8
cagtggtggagtacgtgcctcga

SEQ ID NO: 5 - RNA, 21 nt, synthetic construct
  source 1..21: mol_type = other RNA
  modified_base 1..21: mod_base = OTHER; note = modified as descibed in table 8
agttatcgaggcacatactcc

SEQ ID NO: 6 - RNA, 23 nt, synthetic construct
  source 1..23: mol_type = other RNA
  modified_base 1..23: mod_base = OTHER; note = modified as descibed in table 8
ggagtatgtgcctcgataactct

SEQ ID NO: 7 - RNA, 21 nt, synthetic construct
  source 1..21: mol_type = other RNA
  modified_base 1..2: mod_base = OTHER; note = modified as descibed in table 8
ctgccaagcttggtcatctat

SEQ ID NO: 8 - RNA, 23 nt, synthetic construct
  source 1..23: mol_type = other RNA
  modified_base 1..23: mod_base = OTHER; note = modified as descibed in table 8
atagatgaccaagcttggcaggt

SEQ ID NO: 9 - RNA, 21 nt, synthetic construct
  source 1..21: mol_type = other RNA
  modified_base 1..21: mod_base = OTHER; note = modified as descibed in table 8
cagagttatcgaggcacattc

SEQ ID NO: 10 - RNA, 23 nt, synthetic construct
  source 1..23: mol_type = other RNA
  modified_base 1..23: mod_base = OTHER; note = modified as descibed in table 8
gaatgtgcctcgataactctggc

SEQ ID NO: 11 - RNA, 21 nt, synthetic construct
  source 1..21: mol_type = other RNA
ccggttccaagcctagaggct

SEQ ID NO: 12 - RNA, 23 nt, synthetic construct
  source 1..23: mol_type = other RNA
agcctctaggcttggaaccgggg

SEQ ID NO: 13 - RNA, 21 nt, synthetic construct
  source 1..21: mol_type = other RNA
gttccaagcctagaggctcct

SEQ ID NO: 14 - RNA, 23 nt, synthetic construct
  source 1..23: mol_type = other RNA
aggagcctctaggcttggaaccg

SEQ ID NO: 15 - RNA, 21 nt, synthetic construct
  source 1..21: mol_type = other RNA
aagcctagaggctccttccga

SEQ ID NO: 16 - RNA, 23 nt, synthetic construct
  source 1..23: mol_type = other RNA
tcggaaggagcctctaggcttgg

SEQ ID NO: 17 - RNA, 21 nt, synthetic construct
  source 1..21: mol_type = other RNA
cctagaggctccttccgaaca

SEQ ID NO: 18 - RNA, 23 nt, synthetic construct
  source 1..23: mol_type = other RNA
tgttcggaaggagcctctaggct

SEQ ID NO: 19 - RNA, 21 nt, synthetic construct
  source 1..21: mol_type = other RNA
ctagaggctccttccgaacaa

SEQ ID NO: 20 - RNA, 23 nt, synthetic construct
  source 1..23: mol_type = other RNA
ttgttcggaaggagcctctaggc

SEQ ID NO: 21 - RNA, 21 nt, synthetic construct
  source 1..21: mol_type = other RNA
gaggctccttccgaacaagca

SEQ ID NO: 22 - RNA, 23 nt, synthetic construct
  source 1..23: mol_type = other RNA
tgcttgttcggaaggagcctcta

SEQ ID NO: 23 - RNA, 21 nt, synthetic construct
  source 1..21: mol_type = other RNA
ctccttccgaacaagcaccga

SEQ ID NO: 24 - RNA, 23 nt, synthetic construct
  source 1..23: mol_type = other RNA
tcggtgcttgttcggaaggagcc

SEQ ID NO: 25 - RNA, 21 nt, synthetic construct
  source 1..21: mol_type = other RNA
ttccgaacaagcaccgactga

SEQ ID NO: 26 - RNA, 23 nt, synthetic construct
  source 1..23: mol_type = other RNA
tcagtcggtgcttgttcggaagg

SEQ ID NO: 27 - RNA, 21 nt, synthetic construct
  source 1..21: mol_type = other RNA
cgaacaagcaccgactgagca

SEQ ID NO: 28 - RNA, 23 nt, synthetic construct
  source 1..23: mol_type = other RNA
tgctcagtcggtgcttgttcgga

SEQ ID NO: 29 - RNA, 21 nt, synthetic construct
  source 1..21: mol_type = other RNA
acaagcaccgactgagcaaag

SEQ ID NO: 30 - RNA, 23 nt, synthetic construct
  source 1..23: mol_type = other RNA
ctttgctcagtcggtgcttgttc

SEQ ID NO: 31 - RNA, 21 nt, synthetic construct
  source 1..21: mol_type = other RNA
caagcaccgactgagcaaagg

SEQ ID NO: 32 - RNA, 23 nt, synthetic construct
  source 1..23: mol_type = other RNA
cctttgctcagtcggtgcttgtt

SEQ ID NO: 33 - RNA, 21 nt, synthetic construct
  source 1..21: mol_type = other RNA
gcaccgactgagcaaaggcct

SEQ ID NO: 34 - RNA, 23 nt, synthetic construct
  source 1..23: mol_type = other RNA
aggcctttgctcagtcggtgctt

SEQ ID NO: 35 - RNA, 21 nt, synthetic construct
  source 1..21: mol_type = other RNA
gactgagcaaaggcctggggt

SEQ ID NO: 36 - RNA, 23 nt, synthetic construct
  source 1..23: mol_type = other RNA
accccaggcctttgctcagtcgg

SEQ ID NO: 37 - RNA, 21 nt, synthetic construct
  source 1..21: mol_type = other RNA
aaaggcctggggtgcaggagt

SEQ ID NO: 38 - RNA, 23 nt, synthetic construct
  source 1..23: mol_type = other RNA
actcctgcaccccaggcctttgc

SEQ ID NO: 39 - RNA, 21 nt, synthetic construct
  source 1..21: mol_type = other RNA
ggcctggggtgcaggagtgct

SEQ ID NO: 40 - RNA, 23 nt, synthetic construct
  source 1..23: mol_type = other RNA
agcactcctgcaccccaggcctt

SEQ ID NO: 41 - RNA, 21 nt, synthetic construct
  source 1..21: mol_type = other RNA
ctggggtgcaggagtgctacc

SEQ ID NO: 42 - RNA, 23 nt, synthetic construct
  source 1..23: mol_type = other RNA
ggtagcactcctgcaccccaggc

SEQ ID NO: 43 - RNA, 21 nt, synthetic construct
  source 1..21: mol_type = other RNA
tggggtgcaggagtgctacca

SEQ ID NO: 44 - RNA, 23 nt, synthetic construct
  source 1..23: mol_type = other RNA
tggtagcactcctgcaccccagg

SEQ ID NO: 45 - RNA, 21 nt, synthetic construct
  source 1..21: mol_type = other RNA
ggaagaacctgccaagcttgg

SEQ ID NO: 46 - RNA, 23 nt, synthetic construct
  source 1..23: mol_type = other RNA
ccaagcttggcaggttcttcctg

SEQ ID NO: 47 - RNA, 21 nt, synthetic construct
  source 1..21: mol_type = other RNA
gaagaacctgccaagcttggt

SEQ ID NO: 48 - RNA, 23 nt, synthetic construct
  source 1..23: mol_type = other RNA
accaagcttggcaggttcttcct

SEQ ID NO: 49 - RNA, 21 nt, synthetic construct
  source 1..21: mol_type = other RNA
gaacctgccaagcttggtcat

SEQ ID NO: 50 - RNA, 23 nt, synthetic construct
  source 1..23: mol_type = other RNA
atgaccaagcttggcaggttctt

SEQ ID NO: 51 - RNA, 21 nt, synthetic construct
  source 1..21: mol_type = other RNA
ctgccaagcttggtcatctaa

SEQ ID NO: 52 - RNA, 23 nt, synthetic construct
  source 1..23: mol_type = other RNA
atagatgaccaagcttggcagga

SEQ ID NO: 53 - RNA, 21 nt, synthetic construct
  source 1..21: mol_type = other RNA
caagcttggtcatctatgaca

SEQ ID NO: 54 - RNA, 23 nt, synthetic construct
  source 1..23: mol_type = other RNA
tgtcatagatgaccaagcttggc

SEQ ID NO: 55 - RNA, 21 nt, synthetic construct
  source 1..21: mol_type = other RNA
gcttggtcatctatgacacca

SEQ ID NO: 56 - RNA, 23 nt, synthetic construct
  source 1..23: mol_type = other RNA
tggtgtcatagatgaccaagctt

SEQ ID NO: 57 - RNA, 21 nt, synthetic construct
  source 1..21: mol_type = other RNA
cctagaggctccttccgaaca

SEQ ID NO: 58 - RNA, 23 nt, synthetic construct
  source 1..23: mol_type = other RNA
tgttcggaaggagcctctaggct

SEQ ID NO: 59 - RNA, 21 nt, synthetic construct
  source 1..21: mol_type = other RNA
ctggggtgcaggagtgctacc

SEQ ID NO: 60 - RNA, 23 nt, synthetic construct
  source 1..23: mol_type = other RNA
ggtagcactcctgcaccccaggc

SEQ ID NO: 61 - RNA, 21 nt, synthetic construct
  source 1..21: mol_type = other RNA
gggtgcaggagtgctaccacg

SEQ ID NO: 62 - RNA, 23 nt, synthetic construct
  source 1..23: mol_type = other RNA
cgtggtagcactcctgcacccca

SEQ ID NO: 63 - RNA, 21 nt, synthetic construct
  source 1..21: mol_type = other RNA
gtgcaggagtgctaccacggt

SEQ ID NO: 64 - RNA, 23 nt, synthetic construct
  source 1..23: mol_type = other RNA
accgtggtagcactcctgcaccc

SEQ ID NO: 65 - RNA, 21 nt, synthetic construct
  source 1..21: mol_type = other RNA
caggagtgctaccacggtaat

SEQ ID NO: 66 - RNA, 23 nt, synthetic construct
  source 1..23: mol_type = other RNA
attaccgtggtagcactcctgca

SEQ ID NO: 67 - RNA, 21 nt, synthetic construct
  source 1..21: mol_type = other RNA
taccacggtaatggacagagt

SEQ ID NO: 68 - RNA, 23 nt, synthetic construct
  source 1..23: mol_type = other RNA
actctgtccattaccgtggtagc

SEQ ID NO: 69 - RNA, 21 nt, synthetic construct
  source 1..21: mol_type = other RNA
ccacggtaatggacagagtta

SEQ ID NO: 70 - RNA, 23 nt, synthetic construct
  source 1..23: mol_type = other RNA
taactctgtccattaccgtggta

SEQ ID NO: 71 - RNA, 21 nt, synthetic construct
  source 1..21: mol_type = other RNA
cggtaatggacagagttatcg

SEQ ID NO: 72 - RNA, 23 nt, synthetic construct
  source 1..23: mol_type = other RNA
cgataactctgtccattaccgtg

SEQ ID NO: 73 - RNA, 21 nt, synthetic construct
  source 1..21: mol_type = other RNA
ggtaatggacagagttatcga

SEQ ID NO: 74 - RNA, 23 nt, synthetic construct
  source 1..23: mol_type = other RNA
tcgataactctgtccattaccgt

SEQ ID NO: 75 - RNA, 21 nt, synthetic construct
  source 1..21: mol_type = other RNA
ggacagagttatcgaggcaca

SEQ ID NO: 76 - RNA, 23 nt, synthetic construct
  source 1..23: mol_type = other RNA
tgtgcctcgataactctgtccat

SEQ ID NO: 77 - RNA, 21 nt, synthetic construct
  source 1..21: mol_type = other RNA
gacagagttatcgaggcacat

SEQ ID NO: 78 - RNA, 23 nt, synthetic construct
  source 1..23: mol_type = other RNA
atgtgcctcgataactctgtcca

SEQ ID NO: 79 - RNA, 21 nt, synthetic construct
  source 1..21: mol_type = other RNA
agagttatcgaggcacatact

SEQ ID NO: 80 - RNA, 23 nt, synthetic construct
  source 1..23: mol_type = other RNA
agtatgtgcctcgataactctgt

SEQ ID NO: 81 - RNA, 21 nt, synthetic construct
  source 1..21: mol_type = other RNA
tactgcaggaatccagatcct

SEQ ID NO: 82 - RNA, 23 nt, synthetic construct
  source 1..23: mol_type = other RNA
aggatctggattcctgcagtagt

SEQ ID NO: 83 - RNA, 21 nt, synthetic construct
  source 1..21: mol_type = other RNA
ctgcaggaatccagatcctgt

SEQ ID NO: 84 - RNA, 23 nt, synthetic construct
  source 1..23: mol_type = other RNA
acaggatctggattcctgcagta

SEQ ID NO: 85 - RNA, 21 nt, synthetic construct
  source 1..21: mol_type = other RNA
aggaatccagatcctgtggca

SEQ ID NO: 86 - RNA, 23 nt, synthetic construct
  source 1..23: mol_type = other RNA
tgccacaggatctggattcctgc

SEQ ID NO: 87 - RNA, 21 nt, synthetic construct
  source 1..21: mol_type = other RNA
gaatccagatcctgtggcagc

SEQ ID NO: 88 - RNA, 23 nt, synthetic construct
  source 1..23: mol_type = other RNA
gctgccacaggatctggattcct

SEQ ID NO: 89 - RNA, 21 nt, synthetic construct
  source 1..21: mol_type = other RNA
ccagatcctgtggcagcccct

SEQ ID NO: 90 - RNA, 23 nt, synthetic construct
  source 1..23: mol_type = other RNA
aggggctgccacaggatctggat

SEQ ID NO: 91 - RNA, 21 nt, synthetic construct
  source 1..21: mol_type = other RNA
gatcctgtggcagccccttat

SEQ ID NO: 92 - RNA, 23 nt, synthetic construct
  source 1..23: mol_type = other RNA
ataaggggctgccacaggatctg

SEQ ID NO: 93 - RNA, 21 nt, synthetic construct
  source 1..21: mol_type = other RNA
gtggcagccccttattgttat

SEQ ID NO: 94 - RNA, 23 nt, synthetic construct
  source 1..23: mol_type = other RNA
ataacaataaggggctgccacag

SEQ ID NO: 95 - RNA, 21 nt, synthetic construct
  source 1..21: mol_type = other RNA
ggcagccccttattgttatac

SEQ ID NO: 96 - RNA, 23 nt, synthetic construct
  source 1..23: mol_type = other RNA
gtataacaataaggggctgccac

SEQ ID NO: 97 - RNA, 21 nt, synthetic construct
  source 1..21: mol_type = other RNA
caggtgggagtactgcaacct

SEQ ID NO: 98 - RNA, 23 nt, synthetic construct
  source 1..23: mol_type = other RNA
aggttgcagtactcccacctgac

SEQ ID NO: 99 - RNA, 21 nt, synthetic construct
  source 1..21: mol_type = other RNA
ggtgggagtactgcaacctga

SEQ ID NO: 100 - RNA, 23 nt, synthetic construct
  source 1..23: mol_type = other RNA
tcaggttgcagtactcccacctg

SEQ ID NO: 101 - RNA, 21 nt, synthetic construct
  source 1..21: mol_type = other RNA
agtactgcaacctgacacaat

SEQ ID NO: 102 - RNA, 23 nt, synthetic construct
  source 1..23: mol_type = other RNA
attgtgtcaggttgcagtactcc

SEQ ID NO: 103 - RNA, 21 nt, synthetic construct
  source 1..21: mol_type = other RNA
actgcaacctgacacaatgct

SEQ ID NO: 104 - RNA, 23 nt, synthetic construct
  source 1..23: mol_type = other RNA
agcattgtgtcaggttgcagtac

SEQ ID NO: 105 - RNA, 21 nt, synthetic construct
  source 1..21: mol_type = other RNA
caacctgacacaatgctcaga

SEQ ID NO: 106 - RNA, 23 nt, synthetic construct
  source 1..23: mol_type = other RNA
tctgagcattgtgtcaggttgca

SEQ ID NO: 107 - RNA, 21 nt, synthetic construct
  source 1..21: mol_type = other RNA
ctgacacaatgctcagacgca

SEQ ID NO: 108 - RNA, 23 nt, synthetic construct
  source 1..23: mol_type = other RNA
tgcgtctgagcattgtgtcaggt

SEQ ID NO: 109 - RNA, 21 nt, synthetic construct
  source 1..21: mol_type = other RNA
acacaatgctcagacgcagaa

SEQ ID NO: 110 - RNA, 23 nt, synthetic construct
  source 1..23: mol_type = other RNA
ttctgcgtctgagcattgtgtca

SEQ ID NO: 111 - RNA, 21 nt, synthetic construct
  source 1..21: mol_type = other RNA
tgctcagacgcagaagggact

SEQ ID NO: 112 - RNA, 23 nt, synthetic construct
  source 1..23: mol_type = other RNA
agtcccttctgcgtctgagcatt

SEQ ID NO: 113 - RNA, 21 nt, synthetic construct
  source 1..21: mol_type = other RNA
ctcagacgcagaagggactgc

SEQ ID NO: 114 - RNA, 23 nt, synthetic construct
  source 1..23: mol_type = other RNA
gcagtcccttctgcgtctgagca

SEQ ID NO: 115 - RNA, 21 nt, synthetic construct
  source 1..21: mol_type = other RNA
agacgcagaagggactgccgt

SEQ ID NO: 116 - RNA, 23 nt, synthetic construct
  source 1..23: mol_type = other RNA
acggcagtcccttctgcgtctga

SEQ ID NO: 117 - RNA, 21 nt, synthetic construct
  source 1..21: mol_type = other RNA
ggaagaacctgccaagcttgg

SEQ ID NO: 118 - RNA, 23 nt, synthetic construct
  source 1..23: mol_type = other RNA
ccaagcttggcaggttcttcctg

SEQ ID NO: 119 - RNA, 21 nt, synthetic construct
  source 1..21: mol_type = other RNA
ctgccaagcttggtcatctat

SEQ ID NO: 120 - RNA, 23 nt, synthetic construct
  source 1..23: mol_type = other RNA
atagatgaccaagcttggcaggt

SEQ ID NO: 121 - RNA, 21 nt, synthetic construct
  source 1..21: mol_type = other RNA
caagcttggtcatctatgaca

SEQ ID NO: 122 - RNA, 23 nt, synthetic construct
  source 1..23: mol_type = other RNA
tgtcatagatgaccaagcttggc

SEQ ID NO: 123 - RNA, 21 nt, synthetic construct
  source 1..21: mol_type = other RNA
ggtcatctatgacaccacact

SEQ ID NO: 124 - RNA, 23 nt, synthetic construct
  source 1..23: mol_type = other RNA
agtgtggtgtcatagatgaccaa

SEQ ID NO: 125 - RNA, 21 nt, synthetic construct
  source 1..21: mol_type = other RNA
aactactgccgaaatccagat

SEQ ID NO: 126 - RNA, 23 nt, synthetic construct
  source 1..23: mol_type = other RNA
atctggatttcggcagtagttct

SEQ ID NO: 127 - RNA, 21 nt, synthetic construct
  source 1..21: mol_type = other RNA
ctactgccgaaatccagatcc

SEQ ID NO: 128 - RNA, 23 nt, synthetic construct
  source 1..23: mol_type = other RNA
ggatctggatttcggcagtagtt

SEQ ID NO: 129 - RNA, 21 nt, synthetic construct
  source 1..21: mol_type = other RNA
tactgccgaaatccagatcct

SEQ ID NO: 130 - RNA, 23 nt, synthetic construct
  source 1..23: mol_type = other RNA
aggatctggatttcggcagtagt

SEQ ID NO: 131 - RNA, 21 nt, synthetic construct
  source 1..21: mol_type = other RNA
ctgccgaaatccagatcctgt

SEQ ID NO: 132 - RNA, 23 nt, synthetic construct
  source 1..23: mol_type = other RNA
acaggatctggatttcggcagta

SEQ ID NO: 133 - RNA, 21 nt, synthetic construct
  source 1..21: mol_type = other RNA
cgaaatccagatcctgtggca

SEQ ID NO: 134 - RNA, 23 nt, synthetic construct
  source 1..23: mol_type = other RNA
tgccacaggatctggatttcggc

SEQ ID NO: 135 - RNA, 21 nt, synthetic construct
  source 1..21: mol_type = other RNA
atcctgtggcagccccttggt

SEQ ID NO: 136 - RNA, 23 nt, synthetic construct
  source 1..23: mol_type = other RNA
accaaggggctgccacaggatct

SEQ ID NO: 137 - RNA, 21 nt, synthetic construct
  source 1..21: mol_type = other RNA
ctgtggcagccccttggtgtt

SEQ ID NO: 138 - RNA, 23 nt, synthetic construct
  source 1..23: mol_type = other RNA
aacaccaaggggctgccacagga

SEQ ID NO: 139 - RNA, 21 nt, synthetic construct
  source 1..21: mol_type = other RNA
tggcagccccttggtgttata

SEQ ID NO: 140 - RNA, 23 nt, synthetic construct
  source 1..23: mol_type = other RNA
tataacaccaaggggctgccaca

SEQ ID NO: 141 - RNA, 21 nt, synthetic construct
  source 1..21: mol_type = other RNA
ggcagccccttggtgttatac

SEQ ID NO: 142 - RNA, 23 nt, synthetic construct
  source 1..23: mol_type = other RNA
gtataacaccaaggggctgccac

SEQ ID NO: 143 - RNA, 21 nt, synthetic construct
  source 1..21: mol_type = other RNA
gcagccccttggtgttataca

SEQ ID NO: 144 - RNA, 23 nt, synthetic construct
  source 1..23: mol_type = other RNA
tgtataacaccaaggggctgcca

SEQ ID NO: 145 - RNA, 21 nt, synthetic construct
  source 1..21: mol_type = other RNA
tcccagtgtcaggtgggagta

SEQ ID NO: 146 - RNA, 23 nt, synthetic construct
  source 1..23: mol_type = other RNA
tactcccacctgacactgggatc

SEQ ID NO: 147 - RNA, 21 nt, synthetic construct
  source 1..21: mol_type = other RNA
cccagtgtcaggtgggagtac

SEQ ID NO: 148 - RNA, 23 nt, synthetic construct
  source 1..23: mol_type = other RNA
gtactcccacctgacactgggat

SEQ ID NO: 149 - RNA, 21 nt, synthetic construct
  source 1..21: mol_type = other RNA
ccagtgtcaggtgggagtact

SEQ ID NO: 150 - RNA, 23 nt, synthetic construct
  source 1..23: mol_type = other RNA
agtactcccacctgacactggga

SEQ ID NO: 151 - RNA, 21 nt, synthetic construct
  source 1..21: mol_type = other RNA
tgtcaggtgggagtactgcaa

SEQ ID NO: 152 - RNA, 23 nt, synthetic construct
  source 1..23: mol_type = other RNA
ttgcagtactcccacctgacact

SEQ ID NO: 153 - RNA, 21 nt, synthetic construct
  source 1..21: mol_type = other RNA
ggtgggagtactgcaacctga

SEQ ID NO: 154 - RNA, 23 nt, synthetic construct
  source 1..23: mol_type = other RNA
tcaggttgcagtactcccacctg

SEQ ID NO: 155 - RNA, 21 nt, synthetic construct
  source 1..21: mol_type = other RNA
agtactgcaacctgacacgat

SEQ ID NO: 156 - RNA, 23 nt, synthetic construct
  source 1..23: mol_type = other RNA
atcgtgtcaggttgcagtactcc

SEQ ID NO: 157 - RNA, 21 nt, synthetic construct
  source 1..21: mol_type = other RNA
caacctgacacgatgctcaga

SEQ ID NO: 158 - RNA, 23 nt, synthetic construct
  source 1..23: mol_type = other RNA
tctgagcatcgtgtcaggttgca

SEQ ID NO: 159 - RNA, 21 nt, synthetic construct
  source 1..21: mol_type = other RNA
aacctgacacgatgctcagat

SEQ ID NO: 160 - RNA, 23 nt, synthetic construct
  source 1..23: mol_type = other RNA
atctgagcatcgtgtcaggttgc

SEQ ID NO: 161 - RNA, 21 nt, synthetic construct
  source 1..21: mol_type = other RNA
cctgacacgatgctcagatgc

SEQ ID NO: 162 - RNA, 23 nt, synthetic construct
  source 1..23: mol_type = other RNA
gcatctgagcatcgtgtcaggtt

SEQ ID NO: 163 - RNA, 21 nt, synthetic construct
  source 1..21: mol_type = other RNA
acacgatgctcagatgcagaa

SEQ ID NO: 164 - RNA, 23 nt, synthetic construct
  source 1..23: mol_type = other RNA
ttctgcatctgagcatcgtgtca

SEQ ID NO: 165 - RNA, 21 nt, synthetic construct
  source 1..21: mol_type = other RNA
ggaagaacttgccaagcttgg

SEQ ID NO: 166 - RNA, 23 nt, synthetic construct
  source 1..23: mol_type = other RNA
ccaagcttggcaagttcttcctg

SEQ ID NO: 167 - RNA, 21 nt, synthetic construct
  source 1..21: mol_type = other RNA
gaagaacttgccaagcttggt

SEQ ID NO: 168 - RNA, 23 nt, synthetic construct
  source 1..23: mol_type = other RNA
accaagcttggcaagttcttcct

SEQ ID NO: 169 - RNA, 21 nt, synthetic construct
  source 1..21: mol_type = other RNA
gaacttgccaagcttggtcat

SEQ ID NO: 170 - RNA, 23 nt, synthetic construct
  source 1..23: mol_type = other RNA
atgaccaagcttggcaagttctt

SEQ ID NO: 171 - RNA, 21 nt, synthetic construct
  source 1..21: mol_type = other RNA
ttgccaagcttggtcatctat

SEQ ID NO: 172 - RNA, 23 nt, synthetic construct
  source 1..23: mol_type = other RNA
atagatgaccaagcttggcaagt

SEQ ID NO: 173 - RNA, 21 nt, synthetic construct
  source 1..21: mol_type = other RNA
caagcttggtcatctatgaca

SEQ ID NO: 174 - RNA, 23 nt, synthetic construct
  source 1..23: mol_type = other RNA
tgtcatagatgaccaagcttggc

SEQ ID NO: 175 - RNA, 21 nt, synthetic construct
  source 1..21: mol_type = other RNA
ggtcatctatgacaccacacc

SEQ ID NO: 176 - RNA, 23 nt, synthetic construct
  source 1..23: mol_type = other RNA
ggtgtggtgtcatagatgaccaa

SEQ ID NO: 177 - RNA, 21 nt, synthetic construct
  source 1..21: mol_type = other RNA
tctatgacaccacaccagcat

SEQ ID NO: 178 - RNA, 23 nt, synthetic construct
  source 1..23: mol_type = other RNA
atgctggtgtggtgtcatagatg

SEQ ID NO: 179 - RNA, 21 nt, synthetic construct
  source 1..21: mol_type = other RNA
atgacaccacaccagcatagt

SEQ ID NO: 180 - RNA, 23 nt, synthetic construct
  source 1..23: mol_type = other RNA
actatgctggtgtggtgtcatag

SEQ ID NO: 181 - RNA, 21 nt, synthetic construct
  source 1..21: mol_type = other RNA
caccacaccagcatagtcgga

SEQ ID NO: 182 - RNA, 23 nt, synthetic construct
  source 1..23: mol_type = other RNA
tccgactatgctggtgtggtgtc

SEQ ID NO: 183 - RNA, 21 nt, synthetic construct
  source 1..21: mol_type = other RNA
caccagcatagtcggacccca

SEQ ID NO: 184 - RNA, 23 nt, synthetic construct
  source 1..23: mol_type = other RNA
tggggtccgactatgctggtgtg

SEQ ID NO: 185 - RNA, 21 nt, synthetic construct
  source 1..21: mol_type = other RNA
aaatgctggcctgaccaggaa

SEQ ID NO: 186 - RNA, 23 nt, synthetic construct
  source 1..23: mol_type = other RNA
ttcctggtcaggccagcatttgg

SEQ ID NO: 187 - RNA, 21 nt, synthetic construct
  source 1..21: mol_type = other RNA
gctggcctgaccaggaactac

SEQ ID NO: 188 - RNA, 23 nt, synthetic construct
  source 1..23: mol_type = other RNA
gtagttcctggtcaggccagcat

SEQ ID NO: 189 - RNA, 21 nt, synthetic construct
  source 1..21: mol_type = other RNA
ctggcctgaccaggaactact

SEQ ID NO: 190 - RNA, 23 nt, synthetic construct
  source 1..23: mol_type = other RNA
agtagttcctggtcaggccagca

SEQ ID NO: 191 - RNA, 21 nt, synthetic construct
  source 1..21: mol_type = other RNA
ggcctgaccaggaactactgc

SEQ ID NO: 192 - RNA, 23 nt, synthetic construct
  source 1..23: mol_type = other RNA
gcagtagttcctggtcaggccag

SEQ ID NO: 193 - RNA, 21 nt, synthetic construct
  source 1..21: mol_type = other RNA
ctgaccaggaactactgcagg

SEQ ID NO: 194 - RNA, 23 nt, synthetic construct
  source 1..23: mol_type = other RNA
cctgcagtagttcctggtcaggc

SEQ ID NO: 195 - RNA, 21 nt, synthetic construct
  source 1..21: mol_type = other RNA
gaccaggaactactgcaggaa

SEQ ID NO: 196 - RNA, 23 nt, synthetic construct
  source 1..23: mol_type = other RNA
ttcctgcagtagttcctggtcag

SEQ ID NO: 197 - RNA, 21 nt, synthetic construct
  source 1..21: mol_type = other RNA
ccaggaactactgcaggaatc

SEQ ID NO: 198 - RNA, 23 nt, synthetic construct
  source 1..23: mol_type = other RNA
gattcctgcagtagttcctggtc

SEQ ID NO: 199 - RNA, 21 nt, synthetic construct
  source 1..21: mol_type = other RNA
aactactgcaggaatccagat

SEQ ID NO: 200 - RNA, 23 nt, synthetic construct
  source 1..23: mol_type = other RNA
atctggattcctgcagtagttcc

SEQ ID NO: 201 - RNA, 21 nt, synthetic construct
  source 1..21: mol_type = other RNA
tactgcaggaatccagatgct

SEQ ID NO: 202 - RNA, 23 nt, synthetic construct
  source 1..23: mol_type = other RNA
agcatctggattcctgcagtagt

SEQ ID NO: 203 - RNA, 21 nt, synthetic construct
  source 1..21: mol_type = other RNA
ctgcaggaatccagatgctga

SEQ ID NO: 204 - RNA, 23 nt, synthetic construct
  source 1..23: mol_type = other RNA
tcagcatctggattcctgcagta

SEQ ID NO: 205 - RNA, 21 nt, synthetic construct
  source 1..21: mol_type = other RNA
caggaatccagatgctgagat

SEQ ID NO: 206 - RNA, 23 nt, synthetic construct
  source 1..23: mol_type = other RNA
atctcagcatctggattcctgca

SEQ ID NO: 207 - RNA, 21 nt, synthetic construct
  source 1..21: mol_type = other RNA
ggaatccagatgctgagattc

SEQ ID NO: 208 - RNA, 23 nt, synthetic construct
  source 1..23: mol_type = other RNA
gaatctcagcatctggattcctg

SEQ ID NO: 209 - RNA, 21 nt, synthetic construct
  source 1..21: mol_type = other RNA
gaatccagatgctgagattcg

SEQ ID NO: 210 - RNA, 23 nt, synthetic construct
  source 1..23: mol_type = other RNA
cgaatctcagcatctggattcct

SEQ ID NO: 211 - RNA, 21 nt, synthetic construct
  source 1..21: mol_type = other RNA
cagatgctgagattcgccctt

SEQ ID NO: 212 - RNA, 23 nt, synthetic construct
  source 1..23: mol_type = other RNA
aagggcgaatctcagcatctgga

SEQ ID NO: 213 - RNA, 21 nt, synthetic construct
  source 1..21: mol_type = other RNA
gatgctgagattcgcccttgg

SEQ ID NO: 214 - RNA, 23 nt, synthetic construct
  source 1..23: mol_type = other RNA
ccaagggcgaatctcagcatctg

SEQ ID NO: 215 - RNA, 21 nt, synthetic construct
  source 1..21: mol_type = other RNA
tgagattcgcccttggtgtta

SEQ ID NO: 216 - RNA, 23 nt, synthetic construct
  source 1..23: mol_type = other RNA
taacaccaagggcgaatctcagc

SEQ ID NO: 217 - RNA, 21 nt, synthetic construct
  source 1..21: mol_type = other RNA
atcccagtgtcaggtgggagt

SEQ ID NO: 218 - RNA, 23 nt, synthetic construct
  source 1..23: mol_type = other RNA
actcccacctgacactgggatcc

SEQ ID NO: 219 - RNA, 21 nt, synthetic construct
  source 1..21: mol_type = other RNA
cccagtgtcaggtgggagtac

SEQ ID NO: 220 - RNA, 23 nt, synthetic construct
  source 1..23: mol_type = other RNA
gtactcccacctgacactgggat

SEQ ID NO: 221 - RNA, 21 nt, synthetic construct
  source 1..21: mol_type = other RNA
ggtgggagtactgcaacctga

SEQ ID NO: 222 - RNA, 23 nt, synthetic construct
  source 1..23: mol_type = other RNA
tcaggttgcagtactcccacctg

SEQ ID NO: 223 - RNA, 21 nt, synthetic construct
  source 1..21: mol_type = other RNA
ccatggtgatggacagagtta

SEQ ID NO: 224 - RNA, 23 nt, synthetic construct
  source 1..23: mol_type = other RNA
taactctgtccatcaccatggta

SEQ ID NO: 225 - RNA, 21 nt, synthetic construct
  source 1..21: mol_type = other RNA
ggtgatggacagagttatcga

SEQ ID NO: 226 - RNA, 23 nt, synthetic construct
  source 1..23: mol_type = other RNA
tcgataactctgtccatcaccat

SEQ ID NO: 227 - RNA, 21 nt, synthetic construct
  source 1..21: mol_type = other RNA
atggacagagttatcgaggct

SEQ ID NO: 228 - RNA, 23 nt, synthetic construct
  source 1..23: mol_type = other RNA
agcctcgataactctgtccatca

SEQ ID NO: 229 - RNA, 21 nt, synthetic construct
  source 1..21: mol_type = other RNA
ggacagagttatcgaggctca

SEQ ID NO: 230 - RNA, 23 nt, synthetic construct
  source 1..23: mol_type = other RNA
tgagcctcgataactctgtccat

SEQ ID NO: 231 - RNA, 21 nt, synthetic construct
  source 1..21: mol_type = other RNA
gacagagttatcgaggctcat

SEQ ID NO: 232 - RNA, 23 nt, synthetic construct
  source 1..23: mol_type = other RNA
atgagcctcgataactctgtcca

SEQ ID NO: 233 - RNA, 21 nt, synthetic construct
  source 1..21: mol_type = other RNA
agagttatcgaggctcattct

SEQ ID NO: 234 - RNA, 23 nt, synthetic construct
  source 1..23: mol_type = other RNA
agaatgagcctcgataactctgt

SEQ ID NO: 235 - RNA, 21 nt, synthetic construct
  source 1..21: mol_type = other RNA
cactgtcacaggaaggacatg

SEQ ID NO: 236 - RNA, 23 nt, synthetic construct
  source 1..23: mol_type = other RNA
catgtccttcctgtgacagtggt

SEQ ID NO: 237 - RNA, 21 nt, synthetic construct
  source 1..21: mol_type = other RNA
actgtcacaggaaggacatgt

SEQ ID NO: 238 - RNA, 23 nt, synthetic construct
  source 1..23: mol_type = other RNA
acatgtccttcctgtgacagtgg

SEQ ID NO: 239 - RNA, 21 nt, synthetic construct
  source 1..21: mol_type = other RNA
tcacaggaaggacatgtcagt

SEQ ID NO: 240 - RNA, 23 nt, synthetic construct
  source 1..23: mol_type = other RNA
actgacatgtccttcctgtgaca

SEQ ID NO: 241 - RNA, 21 nt, synthetic construct
  source 1..21: mol_type = other RNA
ggaaggacatgtcagtcttgg

SEQ ID NO: 242 - RNA, 23 nt, synthetic construct
  source 1..23: mol_type = other RNA
ccaagactgacatgtccttcctg

SEQ ID NO: 243 - RNA, 21 nt, synthetic construct
  source 1..21: mol_type = other RNA
gaaggacatgtcagtcttggt

SEQ ID NO: 244 - RNA, 23 nt, synthetic construct
  source 1..23: mol_type = other RNA
accaagactgacatgtccttcct

SEQ ID NO: 245 - RNA, 21 nt, synthetic construct
  source 1..21: mol_type = other RNA
acatgtcagtcttggtcctct

SEQ ID NO: 246 - RNA, 23 nt, synthetic construct
  source 1..23: mol_type = other RNA
agaggaccaagactgacatgtcc

SEQ ID NO: 247 - RNA, 21 nt, synthetic construct
  source 1..21: mol_type = other RNA
gtcagtcttggtcctctatga

SEQ ID NO: 248 - RNA, 23 nt, synthetic construct
  source 1..23: mol_type = other RNA
tcatagaggaccaagactgacat

SEQ ID NO: 249 - RNA, 21 nt, synthetic construct
  source 1..21: mol_type = other RNA
cagtcttggtcctctatgaca

SEQ ID NO: 250 - RNA, 23 nt, synthetic construct
  source 1..23: mol_type = other RNA
tgtcatagaggaccaagactgac

SEQ ID NO: 251 - RNA, 21 nt, synthetic construct
  source 1..21: mol_type = other RNA
tcttggtcctctatgacacca

SEQ ID NO: 252 - RNA, 23 nt, synthetic construct
  source 1..23: mol_type = other RNA
tggtgtcatagaggaccaagact

SEQ ID NO: 253 - RNA, 21 nt, synthetic construct
  source 1..21: mol_type = other RNA
ggtcctctatgacaccacact

SEQ ID NO: 254 - RNA, 23 nt, synthetic construct
  source 1..23: mol_type = other RNA
agtgtggtgtcatagaggaccaa

SEQ ID NO: 255 - RNA, 21 nt, synthetic construct
  source 1..21: mol_type = other RNA
tctatgacaccacactggcat

SEQ ID NO: 256 - RNA, 23 nt, synthetic construct
  source 1..23: mol_type = other RNA
atgccagtgtggtgtcatagagg

SEQ ID NO: 257 - RNA, 21 nt, synthetic construct
  source 1..21: mol_type = other RNA
tgacaccacactggcatcaga

SEQ ID NO: 258 - RNA, 23 nt, synthetic construct
  source 1..23: mol_type = other RNA
tctgatgccagtgtggtgtcata

SEQ ID NO: 259 - RNA, 21 nt, synthetic construct
  source 1..21: mol_type = other RNA
cacactggcatcagaggacaa

SEQ ID NO: 260 - RNA, 23 nt, synthetic construct
  source 1..23: mol_type = other RNA
ttgtcctctgatgccagtgtggt

SEQ ID NO: 261 - RNA, 21 nt, synthetic construct
  source 1..21: mol_type = other RNA
ggcatcagaggacaacagaat

SEQ ID NO: 262 - RNA, 23 nt, synthetic construct
  source 1..23: mol_type = other RNA
attctgttgtcctctgatgccag

SEQ ID NO: 263 - RNA, 21 nt, synthetic construct
  source 1..21: mol_type = other RNA
catcagaggacaacagaatat

SEQ ID NO: 264 - RNA, 23 nt, synthetic construct
  source 1..23: mol_type = other RNA
atattctgttgtcctctgatgcc

SEQ ID NO: 265 - RNA, 21 nt, synthetic construct
  source 1..21: mol_type = other RNA
cagaggacaacagaatattat

SEQ ID NO: 266 - RNA, 23 nt, synthetic construct
  source 1..23: mol_type = other RNA
ataatattctgttgtcctctgat

SEQ ID NO: 267 - RNA, 21 nt, synthetic construct
  source 1..21: mol_type = other RNA
cagaggacaacagaatattat

SEQ ID NO: 268 - RNA, 23 nt, synthetic construct
  source 1..23: mol_type = other RNA
ataatattctgttgtcctctgat

SEQ ID NO: 269 - RNA, 21 nt, synthetic construct
  source 1..21: mol_type = other RNA
gaggacaacagaatattatcc

SEQ ID NO: 270 - RNA, 23 nt, synthetic construct
  source 1..23: mol_type = other RNA
ggataatattctgttgtcctctg

SEQ ID NO: 271 - RNA, 21 nt, synthetic construct
  source 1..21: mol_type = other RNA
ggtggcctgaccaggaactac

SEQ ID NO: 272 - RNA, 23 nt, synthetic construct
  source 1..23: mol_type = other RNA
gtagttcctggtcaggccaccat

SEQ ID NO: 273 - RNA, 21 nt, synthetic construct
  source 1..21: mol_type = other RNA
gtggcctgaccaggaactact

SEQ ID NO: 274 - RNA, 23 nt, synthetic construct
  source 1..23: mol_type = other RNA
agtagttcctggtcaggccacca

SEQ ID NO: 275 - RNA, 21 nt, synthetic construct
  source 1..21: mol_type = other RNA
ggcctgaccaggaactactgc

SEQ ID NO: 276 - RNA, 23 nt, synthetic construct
  source 1..23: mol_type = other RNA
gcagtagttcctggtcaggccac

SEQ ID NO: 277 - RNA, 21 nt, synthetic construct
  source 1..21: mol_type = other RNA
ctgaccaggaactactgcagg

SEQ ID NO: 278 - RNA, 23 nt, synthetic construct
  source 1..23: mol_type = other RNA
cctgcagtagttcctggtcaggc

SEQ ID NO: 279 - RNA, 21 nt, synthetic construct
  source 1..21: mol_type = other RNA
ccaggaactactgcaggaatc

SEQ ID NO: 280 - RNA, 23 nt, synthetic construct
  source 1..23: mol_type = other RNA
gattcctgcagtagttcctggtc

SEQ ID NO: 281 - RNA, 21 nt, synthetic construct
  source 1..21: mol_type = other RNA
ctgcaggaatccagatgctga

SEQ ID NO: 282 - RNA, 23 nt, synthetic construct
  source 1..23: mol_type = other RNA
tcagcatctggattcctgcagta

SEQ ID NO: 283 - RNA, 21 nt, synthetic construct
  source 1..21: mol_type = other RNA
tactgcaacctgacacaatgt

SEQ ID NO: 284 - RNA, 23 nt, synthetic construct
  source 1..23: mol_type = other RNA
acattgtgtcaggttgcagtact

SEQ ID NO: 285 - RNA, 21 nt, synthetic construct
  source 1..21: mol_type = other RNA
caacctgacacaatgtccagt

SEQ ID NO: 286 - RNA, 23 nt, synthetic construct
  source 1..23: mol_type = other RNA
actggacattgtgtcaggttgca

SEQ ID NO: 287 - RNA, 21 nt, synthetic construct
  source 1..21: mol_type = other RNA
ctgacacaatgtccagtgaca

SEQ ID NO: 288 - RNA, 23 nt, synthetic construct
  source 1..23: mol_type = other RNA
tgtcactggacattgtgtcaggt

SEQ ID NO: 289 - RNA, 21 nt, synthetic construct
  source 1..21: mol_type = other RNA
gacacaatgtccagtgacaga

SEQ ID NO: 290 - RNA, 23 nt, synthetic construct
  source 1..23: mol_type = other RNA
tctgtcactggacattgtgtcag

SEQ ID NO: 291 - RNA, 21 nt, synthetic construct
  source 1..21: mol_type = other RNA
cacaatgtccagtgacagaat

SEQ ID NO: 292 - RNA, 23 nt, synthetic construct
  source 1..23: mol_type = other RNA
attctgtcactggacattgtgtc

SEQ ID NO: 293 - RNA, 21 nt, synthetic construct
  source 1..21: mol_type = other RNA
tgtccagtgacagaatcaagt

SEQ ID NO: 294 - RNA, 23 nt, synthetic construct
  source 1..23: mol_type = other RNA
acttgattctgtcactggacatt

SEQ ID NO: 295 - RNA, 21 nt, synthetic construct
  source 1..21: mol_type = other RNA
cagtgacagaatcaagtgtcc

SEQ ID NO: 296 - RNA, 23 nt, synthetic construct
  source 1..23: mol_type = other RNA
ggacacttgattctgtcactgga

SEQ ID NO: 297 - RNA, 21 nt, synthetic construct
  source 1..21: mol_type = other RNA
agtgacagaatcaagtgtcct

SEQ ID NO: 298 - RNA, 23 nt, synthetic construct
  source 1..23: mol_type = other RNA
aggacacttgattctgtcactgg

SEQ ID NO: 299 - RNA, 21 nt, synthetic construct
  source 1..21: mol_type = other RNA
caggactgctaccatggtgat

SEQ ID NO: 300 - RNA, 23 nt, synthetic construct
  source 1..23: mol_type = other RNA
atcaccatggtagcagtcctgga

SEQ ID NO: 301 - RNA, 21 nt, synthetic construct
  source 1..21: mol_type = other RNA
ctgctaccatggtgatggaca

SEQ ID NO: 302 - RNA, 23 nt, synthetic construct
  source 1..23: mol_type = other RNA
tgtccatcaccatggtagcagtc

SEQ ID NO: 303 - RNA, 21 nt, synthetic construct
  source 1..21: mol_type = other RNA
ccatggtgatggacagagtta

SEQ ID NO: 304 - RNA, 23 nt, synthetic construct
  source 1..23: mol_type = other RNA
taactctgtccatcaccatggta

SEQ ID NO: 305 - RNA, 21 nt, synthetic construct
  source 1..21: mol_type = other RNA
ggaaggacatgtcagtcttgg

SEQ ID NO: 306 - RNA, 23 nt, synthetic construct
  source 1..23: mol_type = other RNA
ccaagactgacatgtccttcctg

SEQ ID NO: 307 - RNA, 21 nt, synthetic construct
  source 1..21: mol_type = other RNA
cagtcttggtcctctatgaca

SEQ ID NO: 308 - RNA, 23 nt, synthetic construct
  source 1..23: mol_type = other RNA
tgtcatagaggaccaagactgac

SEQ ID NO: 309 - RNA, 21 nt, synthetic construct
  source 1..21: mol_type = other RNA
ggtcctctatgacaccacact

SEQ ID NO: 310 - RNA, 23 nt, synthetic construct
  source 1..23: mol_type = other RNA
agtgtggtgtcatagaggaccaa

SEQ ID NO: 311 - RNA, 21 nt, synthetic construct
  source 1..21: mol_type = other RNA
ctgcaggaatccagatgctga

SEQ ID NO: 312 - RNA, 23 nt, synthetic construct
  source 1..23: mol_type = other RNA
tcagcatctggattcctgcagta

SEQ ID NO: 313 - RNA, 21 nt, synthetic construct
  source 1..21: mol_type = other RNA
ggaatccagatgctgagattc

SEQ ID NO: 314 - RNA, 23 nt, synthetic construct
  source 1..23: mol_type = other RNA
gaatctcagcatctggattcctg

SEQ ID NO: 315 - RNA, 21 nt, synthetic construct
  source 1..21: mol_type = other RNA
gaatccagatgctgagattcg

SEQ ID NO: 316 - RNA, 23 nt, synthetic construct
  source 1..23: mol_type = other RNA
cgaatctcagcatctggattcct

SEQ ID NO: 317 - RNA, 21 nt, synthetic construct
  source 1..21: mol_type = other RNA
gatgctgagattcgcccttgg

SEQ ID NO: 318 - RNA, 23 nt, synthetic construct
  source 1..23: mol_type = other RNA
ccaagggcgaatctcagcatctg

SEQ ID NO: 319 - RNA, 21 nt, synthetic construct
  source 1..21: mol_type = other RNA
gagattcgcccttggtgttat

SEQ ID NO: 320 - RNA, 23 nt, synthetic construct
  source 1..23: mol_type = other RNA
ataacaccaagggcgaatctcag

SEQ ID NO: 321 - RNA, 21 nt, synthetic construct
  source 1..21: mol_type = other RNA
gattcgcccttggtgttatac

SEQ ID NO: 322 - RNA, 23 nt, synthetic construct
  source 1..23: mol_type = other RNA
gtataacaccaagggcgaatctc

SEQ ID NO: 323 - RNA, 21 nt, synthetic construct
  source 1..21: mol_type = other RNA
tcgcccttggtgttataccat

SEQ ID NO: 324 - RNA, 23 nt, synthetic construct
  source 1..23: mol_type = other RNA
atggtataacaccaagggcgaat

SEQ ID NO: 325 - RNA, 21 nt, synthetic construct
  source 1..21: mol_type = other RNA
cgcccttggtgttataccatg

SEQ ID NO: 326 - RNA, 23 nt, synthetic construct
  source 1..23: mol_type = other RNA
catggtataacaccaagggcgaa

SEQ ID NO: 327 - RNA, 21 nt, synthetic construct
  source 1..21: mol_type = other RNA
ccttggtgttataccatggat

SEQ ID NO: 328 - RNA, 23 nt, synthetic construct
  source 1..23: mol_type = other RNA
atccatggtataacaccaagggc

SEQ ID NO: 329 - RNA, 21 nt, synthetic construct
  source 1..21: mol_type = other RNA
cttggtgttataccatggatc

SEQ ID NO: 330 - RNA, 23 nt, synthetic construct
  source 1..23: mol_type = other RNA
gatccatggtataacaccaaggg

SEQ ID NO: 331 - RNA, 21 nt, synthetic construct
  source 1..21: mol_type = other RNA
ggtgttataccatggatccca

SEQ ID NO: 332 - RNA, 23 nt, synthetic construct
  source 1..23: mol_type = other RNA
tgggatccatggtataacaccaa

SEQ ID NO: 333 - RNA, 21 nt, synthetic construct
  source 1..21: mol_type = other RNA
gatgctgagattcgcccttgg

SEQ ID NO: 334 - RNA, 23 nt, synthetic construct
  source 1..23: mol_type = other RNA
ccaagggcgaatctcagcatctg

SEQ ID NO: 335 - RNA, 21 nt, synthetic construct
  source 1..21: mol_type = other RNA
agattcgcccttggtgttaca

SEQ ID NO: 336 - RNA, 23 nt, synthetic construct
  source 1..23: mol_type = other RNA
tgtaacaccaagggcgaatctca

SEQ ID NO: 337 - RNA, 21 nt, synthetic construct
  source 1..21: mol_type = other RNA
tcgcccttggtgttacaccat

SEQ ID NO: 338 - RNA, 23 nt, synthetic construct
  source 1..23: mol_type = other RNA
atggtgtaacaccaagggcgaat

SEQ ID NO: 339 - RNA, 21 nt, synthetic construct
  source 1..21: mol_type = other RNA
cgcccttggtgttacaccatg

SEQ ID NO: 340 - RNA, 23 nt, synthetic construct
  source 1..23: mol_type = other RNA
catggtgtaacaccaagggcgaa

SEQ ID NO: 341 - RNA, 21 nt, synthetic construct
  source 1..21: mol_type = other RNA
ccttggtgttacaccatggat

SEQ ID NO: 342 - RNA, 23 nt, synthetic construct
  source 1..23: mol_type = other RNA
atccatggtgtaacaccaagggc

SEQ ID NO: 343 - RNA, 21 nt, synthetic construct
  source 1..21: mol_type = other RNA
cttggtgttacaccatggatc

SEQ ID NO: 344 - RNA, 23 nt, synthetic construct
  source 1..23: mol_type = other RNA
gatccatggtgtaacaccaaggg

SEQ ID NO: 345 - RNA, 21 nt, synthetic construct
  source 1..21: mol_type = other RNA
tgttacaccatggatcccagt

SEQ ID NO: 346 - RNA, 23 nt, synthetic construct
  source 1..23: mol_type = other RNA
actgggatccatggtgtaacacc

SEQ ID NO: 347 - RNA, 21 nt, synthetic construct
  source 1..21: mol_type = other RNA
acaccatggatcccagtgtca

SEQ ID NO: 348 - RNA, 23 nt, synthetic construct
  source 1..23: mol_type = other RNA
tgacactgggatccatggtgtaa

SEQ ID NO: 349 - RNA, 21 nt, synthetic construct
  source 1..21: mol_type = other RNA
ccatggatcccagtgtcaggt

SEQ ID NO: 350 - RNA, 23 nt, synthetic construct
  source 1..23: mol_type = other RNA
acctgacactgggatccatggtg

SEQ ID NO: 351 - RNA, 21 nt, synthetic construct
  source 1..21: mol_type = other RNA
cccagtgtcaggtgggagtac

SEQ ID NO: 352 - RNA, 23 nt, synthetic construct
  source 1..23: mol_type = other RNA
gtactcccacctgacactgggat

SEQ ID NO: 353 - RNA, 21 nt, synthetic construct
  source 1..21: mol_type = other RNA
ggtgggagtactgcaacctga

SEQ ID NO: 354 - RNA, 23 nt, synthetic construct
  source 1..23: mol_type = other RNA
tcaggttgcagtactcccacctg

SEQ ID NO: 355 - RNA, 21 nt, synthetic construct
  source 1..21: mol_type = other RNA
ttccaagcacagaggctcctt

SEQ ID NO: 356 - RNA, 23 nt, synthetic construct
  source 1..23: mol_type = other RNA
aaggagcctctgtgcttggaacc

SEQ ID NO: 357 - RNA, 21 nt, synthetic construct
  source 1..21: mol_type = other RNA
agcacagaggctccttctgaa

SEQ ID NO: 358 - RNA, 23 nt, synthetic construct
  source 1..23: mol_type = other RNA
ttcagaaggagcctctgtgcttg

SEQ ID NO: 359 - RNA, 21 nt, synthetic construct
  source 1..21: mol_type = other RNA
cacagaggctccttctgaaca

SEQ ID NO: 360 - RNA, 23 nt, synthetic construct
  source 1..23: mol_type = other RNA
tgttcagaaggagcctctgtgct

SEQ ID NO: 361 - RNA, 21 nt, synthetic construct
  source 1..21: mol_type = other RNA
gaggctccttctgaacaagca

SEQ ID NO: 362 - RNA, 23 nt, synthetic construct
  source 1..23: mol_type = other RNA
tgcttgttcagaaggagcctctg

SEQ ID NO: 363 - RNA, 21 nt, synthetic construct
  source 1..21: mol_type = other RNA
ggctccttctgaacaagcacc

SEQ ID NO: 364 - RNA, 23 nt, synthetic construct
  source 1..23: mol_type = other RNA
ggtgcttgttcagaaggagcctc

SEQ ID NO: 365 - RNA, 21 nt, synthetic construct
  source 1..21: mol_type = other RNA
ccttctgaacaagcaccacct

SEQ ID NO: 366 - RNA, 23 nt, synthetic construct
  source 1..23: mol_type = other RNA
aggtggtgcttgttcagaaggag

SEQ ID NO: 367 - RNA, 21 nt, synthetic construct
  source 1..21: mol_type = other RNA
tgaacaagcaccacctgagaa

SEQ ID NO: 368 - RNA, 23 nt, synthetic construct
  source 1..23: mol_type = other RNA
ttctcaggtggtgcttgttcaga

SEQ ID NO: 369 - RNA, 21 nt, synthetic construct
  source 1..21: mol_type = other RNA
gcaccacctgagaaaagccct

SEQ ID NO: 370 - RNA, 23 nt, synthetic construct
  source 1..23: mol_type = other RNA
agggcttttctcaggtggtgctt

SEQ ID NO: 371 - RNA, 21 nt, synthetic construct
  source 1..21: mol_type = other RNA
cacctgagaaaagccctgtgg

SEQ ID NO: 372 - RNA, 23 nt, synthetic construct
  source 1..23: mol_type = other RNA
ccacagggcttttctcaggtggt

SEQ ID NO: 373 - RNA, 21 nt, synthetic construct
  source 1..21: mol_type = other RNA
acctgagaaaagccctgtggt

SEQ ID NO: 374 - RNA, 23 nt, synthetic construct
  source 1..23: mol_type = other RNA
accacagggcttttctcaggtgg

SEQ ID NO: 375 - RNA, 21 nt, synthetic construct
  source 1..21: mol_type = other RNA
aaaagccctgtggtccaggat

SEQ ID NO: 376 - RNA, 23 nt, synthetic construct
  source 1..23: mol_type = other RNA
atcctggaccacagggcttttct

SEQ ID NO: 377 - RNA, 21 nt, synthetic construct
  source 1..21: mol_type = other RNA
ccctgtggtccaggattgcta

SEQ ID NO: 378 - RNA, 23 nt, synthetic construct
  source 1..23: mol_type = other RNA
tagcaatcctggaccacagggct

SEQ ID NO: 379 - RNA, 21 nt, synthetic construct
  source 1..21: mol_type = other RNA
ctgtggtccaggattgctacc

SEQ ID NO: 380 - RNA, 23 nt, synthetic construct
  source 1..23: mol_type = other RNA
ggtagcaatcctggaccacaggg

SEQ ID NO: 381 - RNA, 21 nt, synthetic construct
  source 1..21: mol_type = other RNA
gtggtccaggattgctaccat

SEQ ID NO: 382 - RNA, 23 nt, synthetic construct
  source 1..23: mol_type = other RNA
atggtagcaatcctggaccacag

SEQ ID NO: 383 - RNA, 21 nt, synthetic construct
  source 1..21: mol_type = other RNA
ggtccaggattgctaccatgg

SEQ ID NO: 384 - RNA, 23 nt, synthetic construct
  source 1..23: mol_type = other RNA
ccatggtagcaatcctggaccac

SEQ ID NO: 385 - RNA, 21 nt, synthetic construct
  source 1..21: mol_type = other RNA
caggattgctaccatggtgat

SEQ ID NO: 386 - RNA, 23 nt, synthetic construct
  source 1..23: mol_type = other RNA
atcaccatggtagcaatcctgga

SEQ ID NO: 387 - RNA, 21 nt, synthetic construct
  source 1..21: mol_type = other RNA
ggtcatctatgataccacact

SEQ ID NO: 388 - RNA, 23 nt, synthetic construct
  source 1..23: mol_type = other RNA
agtgtggtatcatagatgaccaa

SEQ ID NO: 389 - RNA, 21 nt, synthetic construct
  source 1..21: mol_type = other RNA
tctatgataccacactggcat

SEQ ID NO: 390 - RNA, 23 nt, synthetic construct
  source 1..23: mol_type = other RNA
atgccagtgtggtatcatagatg

SEQ ID NO: 391 - RNA, 21 nt, synthetic construct
  source 1..21: mol_type = other RNA
taccacactggcatcagagga

SEQ ID NO: 392 - RNA, 23 nt, synthetic construct
  source 1..23: mol_type = other RNA
tcctctgatgccagtgtggtatc

SEQ ID NO: 393 - RNA, 21 nt, synthetic construct
  source 1..21: mol_type = other RNA
tggcatcagaggaccccagaa

SEQ ID NO: 394 - RNA, 23 nt, synthetic construct
  source 1..23: mol_type = other RNA
ttctggggtcctctgatgccagt

SEQ ID NO: 395 - RNA, 21 nt, synthetic construct
  source 1..21: mol_type = other RNA
catcagaggaccccagaaaac

SEQ ID NO: 396 - RNA, 23 nt, synthetic construct
  source 1..23: mol_type = other RNA
gttttctggggtcctctgatgcc

SEQ ID NO: 397 - RNA, 21 nt, synthetic construct
  source 1..21: mol_type = other RNA
atcagaggaccccagaaaact

SEQ ID NO: 398 - RNA, 23 nt, synthetic construct
  source 1..23: mol_type = other RNA
agttttctggggtcctctgatgc

SEQ ID NO: 399 - RNA, 21 nt, synthetic construct
  source 1..21: mol_type = other RNA
gaccccagaaaactacccaaa

SEQ ID NO: 400 - RNA, 23 nt, synthetic construct
  source 1..23: mol_type = other RNA
tttgggtagttttctggggtcct

SEQ ID NO: 401 - RNA, 21 nt, synthetic construct
  source 1..21: mol_type = other RNA
accccagaaaactacccaaat

SEQ ID NO: 402 - RNA, 23 nt, synthetic construct
  source 1..23: mol_type = other RNA
atttgggtagttttctggggtcc

SEQ ID NO: 403 - RNA, 21 nt, synthetic construct
  source 1..21: mol_type = other RNA
ccccagaaaactacccaaatg

SEQ ID NO: 404 - RNA, 23 nt, synthetic construct
  source 1..23: mol_type = other RNA
catttgggtagttttctggggtc

SEQ ID NO: 405 - RNA, 21 nt, synthetic construct
  source 1..21: mol_type = other RNA
aaactacccaaatgctggcct

SEQ ID NO: 406 - RNA, 23 nt, synthetic construct
  source 1..23: mol_type = other RNA
aggccagcatttgggtagttttc

SEQ ID NO: 407 - RNA, 21 nt, synthetic construct
  source 1..21: mol_type = other RNA
actactgcaggaatccagatt

SEQ ID NO: 408 - RNA, 23 nt, synthetic construct
  source 1..23: mol_type = other RNA
aatctggattcctgcagtagttc

SEQ ID NO: 409 - RNA, 21 nt, synthetic construct
  source 1..21: mol_type = other RNA
tactgcaggaatccagattct

SEQ ID NO: 410 - RNA, 23 nt, synthetic construct
  source 1..23: mol_type = other RNA
agaatctggattcctgcagtagt

SEQ ID NO: 411 - RNA, 21 nt, synthetic construct
  source 1..21: mol_type = other RNA
ctgcaggaatccagattctgg

SEQ ID NO: 412 - RNA, 23 nt, synthetic construct
  source 1..23: mol_type = other RNA
ccagaatctggattcctgcagta

SEQ ID NO: 413 - RNA, 21 nt, synthetic construct
  source 1..21: mol_type = other RNA
caggaatccagattctgggaa

SEQ ID NO: 414 - RNA, 23 nt, synthetic construct
  source 1..23: mol_type = other RNA
ttcccagaatctggattcctgca

SEQ ID NO: 415 - RNA, 21 nt, synthetic construct
  source 1..21: mol_type = other RNA
ggaatccagattctgggaaac

SEQ ID NO: 416 - RNA, 23 nt, synthetic construct
  source 1..23: mol_type = other RNA
gtttcccagaatctggattcctg

SEQ ID NO: 417 - RNA, 21 nt, synthetic construct
  source 1..21: mol_type = other RNA
gaatccagattctgggaaaca

SEQ ID NO: 418 - RNA, 23 nt, synthetic construct
  source 1..23: mol_type = other RNA
tgtttcccagaatctggattcct

SEQ ID NO: 419 - RNA, 21 nt, synthetic construct
  source 1..21: mol_type = other RNA
cagattctgggaaacaaccct

SEQ ID NO: 420 - RNA, 23 nt, synthetic construct
  source 1..23: mol_type = other RNA
agggttgtttcccagaatctgga

SEQ ID NO: 421 - RNA, 21 nt, synthetic construct
  source 1..21: mol_type = other RNA
gattctgggaaacaaccctgg

SEQ ID NO: 422 - RNA, 23 nt, synthetic construct
  source 1..23: mol_type = other RNA
ccagggttgtttcccagaatctg

SEQ ID NO: 423 - RNA, 21 nt, synthetic construct
  source 1..21: mol_type = other RNA
tctgggaaacaaccctggtgt

SEQ ID NO: 424 - RNA, 23 nt, synthetic construct
  source 1..23: mol_type = other RNA
acaccagggttgtttcccagaat

SEQ ID NO: 425 - RNA, 21 nt, synthetic construct
  source 1..21: mol_type = other RNA
acacaatgctcagaaacagaa

SEQ ID NO: 426 - RNA, 23 nt, synthetic construct
  source 1..23: mol_type = other RNA
ttctgtttctgagcattgtgtca

SEQ ID NO: 427 - RNA, 21 nt, synthetic construct
  source 1..21: mol_type = other RNA
tgctcagaaacagaatcaggt

SEQ ID NO: 428 - RNA, 23 nt, synthetic construct
  source 1..23: mol_type = other RNA
acctgattctgtttctgagcatt

SEQ ID NO: 429 - RNA, 21 nt, synthetic construct
  source 1..21: mol_type = other RNA
ctcagaaacagaatcaggtgt

SEQ ID NO: 430 - RNA, 23 nt, synthetic construct
  source 1..23: mol_type = other RNA
acacctgattctgtttctgagca

SEQ ID NO: 431 - RNA, 21 nt, synthetic construct
  source 1..21: mol_type = other RNA
cagaaacagaatcaggtgtcc

SEQ ID NO: 432 - RNA, 23 nt, synthetic construct
  source 1..23: mol_type = other RNA
ggacacctgattctgtttctgag

SEQ ID NO: 433 - RNA, 21 nt, synthetic construct
  source 1..21: mol_type = other RNA
agaaacagaatcaggtgtcct

SEQ ID NO: 434 - RNA, 23 nt, synthetic construct
  source 1..23: mol_type = other RNA
aggacacctgattctgtttctga

SEQ ID NO: 435 - RNA, 21 nt, synthetic construct
  source 1..21: mol_type = other RNA
gaatcaggtgtcctagagact

SEQ ID NO: 436 - RNA, 23 nt, synthetic construct
  source 1..23: mol_type = other RNA
agtctctaggacacctgattctg

SEQ ID NO: 437 - RNA, 21 nt, synthetic construct
  source 1..21: mol_type = other RNA
ggtgtcctagagactcccact

SEQ ID NO: 438 - RNA, 23 nt, synthetic construct
  source 1..23: mol_type = other RNA
agtgggagtctctaggacacctg

SEQ ID NO: 439 - RNA, 21 nt, synthetic construct
  source 1..21: mol_type = other RNA
cctagagactcccactgttgt

SEQ ID NO: 440 - RNA, 23 nt, synthetic construct
  source 1..23: mol_type = other RNA
acaacagtgggagtctctaggac

SEQ ID NO: 441 - RNA, 21 nt, synthetic construct
  source 1..21: mol_type = other RNA
gagttatcgaggcacattctc

SEQ ID NO: 442 - RNA, 23 nt, synthetic construct
  source 1..23: mol_type = other RNA
gagaatgtgcctcgataactctg

SEQ ID NO: 443 - RNA, 21 nt, synthetic construct
  source 1..21: mol_type = other RNA
cgaggcacattctccaccact

SEQ ID NO: 444 - RNA, 23 nt, synthetic construct
  source 1..23: mol_type = other RNA
agtggtggagaatgtgcctcgat

SEQ ID NO: 445 - RNA, 21 nt, synthetic construct
  source 1..21: mol_type = other RNA
tctccaccactgtcacaggaa

SEQ ID NO: 446 - RNA, 23 nt, synthetic construct
  source 1..23: mol_type = other RNA
ttcctgtgacagtggtggagaat

SEQ ID NO: 447 - RNA, 21 nt, synthetic construct
  source 1..21: mol_type = other RNA
ctccaccactgtcacaggaag

SEQ ID NO: 448 - RNA, 23 nt, synthetic construct
  source 1..23: mol_type = other RNA
cttcctgtgacagtggtggagaa

SEQ ID NO: 449 - RNA, 21 nt, synthetic construct
  source 1..21: mol_type = other RNA
ccactgtcacaggaaggacat

SEQ ID NO: 450 - RNA, 23 nt, synthetic construct
  source 1..23: mol_type = other RNA
atgtccttcctgtgacagtggtg

SEQ ID NO: 451 - RNA, 21 nt, synthetic construct
  source 1..21: mol_type = other RNA
cactgtcacaggaaggacatg

SEQ ID NO: 452 - RNA, 23 nt, synthetic construct
  source 1..23: mol_type = other RNA
catgtccttcctgtgacagtggt

SEQ ID NO: 453 - RNA, 21 nt, synthetic construct
  source 1..21: mol_type = other RNA
ggaaggacatgtcaatcttgg

SEQ ID NO: 454 - RNA, 23 nt, synthetic construct
  source 1..23: mol_type = other RNA
ccaagattgacatgtccttcctg

SEQ ID NO: 455 - RNA, 21 nt, synthetic construct
  source 1..21: mol_type = other RNA
gaaggacatgtcaatcttggt

SEQ ID NO: 456 - RNA, 23 nt, synthetic construct
  source 1..23: mol_type = other RNA
accaagattgacatgtccttcct

SEQ ID NO: 457 - RNA, 21 nt, synthetic construct
  source 1..21: mol_type = other RNA
gacatgtcaatcttggtcatc

SEQ ID NO: 458 - RNA, 23 nt, synthetic construct
  source 1..23: mol_type = other RNA
gatgaccaagattgacatgtcct

SEQ ID NO: 459 - RNA, 21 nt, synthetic construct
  source 1..21: mol_type = other RNA
atgtcaatcttggtcatccat

SEQ ID NO: 460 - RNA, 23 nt, synthetic construct
  source 1..23: mol_type = other RNA
atggatgaccaagattgacatgt

SEQ ID NO: 461 - RNA, 21 nt, synthetic construct
  source 1..21: mol_type = other RNA
caatcttggtcatccatgaca

SEQ ID NO: 462 - RNA, 23 nt, synthetic construct
  source 1..23: mol_type = other RNA
tgtcatggatgaccaagattgac

SEQ ID NO: 463 - RNA, 21 nt, synthetic construct
  source 1..21: mol_type = other RNA
ttggtcatccatgacaccaca

SEQ ID NO: 464 - RNA, 23 nt, synthetic construct
  source 1..23: mol_type = other RNA
tgtggtgtcatggatgaccaaga

SEQ ID NO: 465 - RNA, 21 nt, synthetic construct
  source 1..21: mol_type = other RNA
ggtcatccatgacaccacacc

SEQ ID NO: 466 - RNA, 23 nt, synthetic construct
  source 1..23: mol_type = other RNA
ggtgtggtgtcatggatgaccaa

SEQ ID NO: 467 - RNA, 21 nt, synthetic construct
  source 1..21: mol_type = other RNA
agtactgcaacctgacgcgat

SEQ ID NO: 468 - RNA, 23 nt, synthetic construct
  source 1..23: mol_type = other RNA
atcgcgtcaggttgcagtactcc

SEQ ID NO: 469 - RNA, 21 nt, synthetic construct
  source 1..21: mol_type = other RNA
actgcaacctgacgcgatgct

SEQ ID NO: 470 - RNA, 23 nt, synthetic construct
  source 1..23: mol_type = other RNA
agcatcgcgtcaggttgcagtac

SEQ ID NO: 471 - RNA, 21 nt, synthetic construct
  source 1..21: mol_type = other RNA
ctgacgcgatgctcagacaca

SEQ ID NO: 472 - RNA, 23 nt, synthetic construct
  source 1..23: mol_type = other RNA
tgtgtctgagcatcgcgtcaggt

SEQ ID NO: 473 - RNA, 21 nt, synthetic construct
  source 1..21: mol_type = other RNA
acgcgatgctcagacacagaa

SEQ ID NO: 474 - RNA, 23 nt, synthetic construct
  source 1..23: mol_type = other RNA
ttctgtgtctgagcatcgcgtca

SEQ ID NO: 475 - RNA, 21 nt, synthetic construct
  source 1..21: mol_type = other RNA
gcgatgctcagacacagaagg

SEQ ID NO: 476 - RNA, 23 nt, synthetic construct
  source 1..23: mol_type = other RNA
ccttctgtgtctgagcatcgcgt

SEQ ID NO: 477 - RNA, 21 nt, synthetic construct
  source 1..21: mol_type = other RNA
tgctcagacacagaagggact

SEQ ID NO: 478 - RNA, 23 nt, synthetic construct
  source 1..23: mol_type = other RNA
agtcccttctgtgtctgagcatc

SEQ ID NO: 479 - RNA, 21 nt, synthetic construct
  source 1..21: mol_type = other RNA
ctcagacacagaagggactgt

SEQ ID NO: 480 - RNA, 23 nt, synthetic construct
  source 1..23: mol_type = other RNA
acagtcccttctgtgtctgagca

SEQ ID NO: 481 - RNA, 21 nt, synthetic construct
  source 1..21: mol_type = other RNA
cagacacagaagggactgtgg

SEQ ID NO: 482 - RNA, 23 nt, synthetic construct
  source 1..23: mol_type = other RNA
ccacagtcccttctgtgtctgag

SEQ ID NO: 483 - RNA, 21 nt, synthetic construct
  source 1..21: mol_type = other RNA
agacacagaagggactgtggt

SEQ ID NO: 484 - RNA, 23 nt, synthetic construct
  source 1..23: mol_type = other RNA
accacagtcccttctgtgtctga

SEQ ID NO: 485 - RNA, 21 nt, synthetic construct
  source 1..21: mol_type = other RNA
agagttatcgaggcacgtact

SEQ ID NO: 486 - RNA, 23 nt, synthetic construct
  source 1..23: mol_type = other RNA
agtacgtgcctcgataactctgt

SEQ ID NO: 487 - RNA, 21 nt, synthetic construct
  source 1..21: mol_type = other RNA
gagttatcgaggcacgtactc

SEQ ID NO: 488 - RNA, 23 nt, synthetic construct
  source 1..23: mol_type = other RNA
gagtacgtgcctcgataactctg

SEQ ID NO: 489 - RNA, 21 nt, synthetic construct
  source 1..21: mol_type = other RNA
agttatcgaggcacgtactcc

SEQ ID NO: 490 - RNA, 23 nt, synthetic construct
  source 1..23: mol_type = other RNA
ggagtacgtgcctcgataactct

SEQ ID NO: 491 - RNA, 21 nt, synthetic construct
  source 1..21: mol_type = other RNA
gaggcacgtactccaccactg

SEQ ID NO: 492 - RNA, 23 nt, synthetic construct
  source 1..23: mol_type = other RNA
cagtggtggagtacgtgcctcga

SEQ ID NO: 493 - RNA, 21 nt, synthetic construct
  source 1..21: mol_type = other RNA
gacaccacatcaacataatag

SEQ ID NO: 494 - RNA, 23 nt, synthetic construct
  source 1..23: mol_type = other RNA
ctattatgttgatgtggtgtcat

SEQ ID NO: 495 - RNA, 21 nt, synthetic construct
  source 1..21: mol_type = other RNA
acaccacatcaacataatagg

SEQ ID NO: 496 - RNA, 23 nt, synthetic construct
  source 1..23: mol_type = other RNA
cctattatgttgatgtggtgtca

SEQ ID NO: 497 - RNA, 21 nt, synthetic construct
  source 1..21: mol_type = other RNA
accacatcaacataataggac

SEQ ID NO: 498 - RNA, 23 nt, synthetic construct
  source 1..23: mol_type = other RNA
gtcctattatgttgatgtggtgt

SEQ ID NO: 499 - RNA, 21 nt, synthetic construct
  source 1..21: mol_type = other RNA
gctgtggcagctccttattgt

SEQ ID NO: 500 - RNA, 23 nt, synthetic construct
  source 1..23: mol_type = other RNA
acaataaggagctgccacagcat

SEQ ID NO: 501 - RNA, 21 nt, synthetic construct
  source 1..21: mol_type = other RNA
cagctccttattgttatacga

SEQ ID NO: 502 - RNA, 23 nt, synthetic construct
  source 1..23: mol_type = other RNA
tcgtataacaataaggagctgcc

SEQ ID NO: 503 - RNA, 21 nt, synthetic construct
  source 1..21: mol_type = other RNA
agctccttattgttatacgag

SEQ ID NO: 504 - RNA, 23 nt, synthetic construct
  source 1..23: mol_type = other RNA
ctcgtataacaataaggagctgc

SEQ ID NO: 505 - RNA, 21 nt, synthetic construct
  source 1..21: mol_type = other RNA
ttattgttatacgagggatcc

SEQ ID NO: 506 - RNA, 23 nt, synthetic construct
  source 1..23: mol_type = other RNA
ggatccctcgtataacaataagg

SEQ ID NO: 507 - RNA, 21 nt, synthetic construct
  source 1..21: mol_type = other RNA
attgttatacgagggatcccg

SEQ ID NO: 508 - RNA, 23 nt, synthetic construct
  source 1..23: mol_type = other RNA
cgggatccctcgtataacaataa

SEQ ID NO: 509 - RNA, 21 nt, synthetic construct
  source 1..21: mol_type = other RNA
ttgttatacgagggatcccgg

SEQ ID NO: 510 - RNA, 23 nt, synthetic construct
  source 1..23: mol_type = other RNA
ccgggatccctcgtataacaata

SEQ ID NO: 511 - RNA, 21 nt, synthetic construct
  source 1..21: mol_type = other RNA
gttatacgagggatcccggtg

SEQ ID NO: 512 - RNA, 23 nt, synthetic construct
  source 1..23: mol_type = other RNA
caccgggatccctcgtataacaa

SEQ ID NO: 513 - RNA, 21 nt, synthetic construct
  source 1..21: mol_type = other RNA
gagggatcccggtgtcaggtg

SEQ ID NO: 514 - RNA, 23 nt, synthetic construct
  source 1..23: mol_type = other RNA
cacctgacaccgggatccctcgt

SEQ ID NO: 515 - RNA, 21 nt, synthetic construct
  source 1..21: mol_type = other RNA
ctgcaacctgacgcaatgctc

SEQ ID NO: 516 - RNA, 23 nt, synthetic construct
  source 1..23: mol_type = other RNA
gagcattgcgtcaggttgcagta

SEQ ID NO: 517 - RNA, 21 nt, synthetic construct
  source 1..21: mol_type = other RNA
aacctgacgcaatgctcagac

SEQ ID NO: 518 - RNA, 23 nt, synthetic construct
  source 1..23: mol_type = other RNA
gtctgagcattgcgtcaggttgc

SEQ ID NO: 519 - RNA, 21 nt, synthetic construct
  source 1..21: mol_type = other RNA
gaagggactgccgtcgcgcct

SEQ ID NO: 520 - RNA, 23 nt, synthetic construct
  source 1..23: mol_type = other RNA
aggcgcgacggcagtcccttctg

SEQ ID NO: 521 - RNA, 21 nt, synthetic construct
  source 1..21: mol_type = other RNA
cgtcgcgcctccgactgttac

SEQ ID NO: 522 - RNA, 23 nt, synthetic construct
  source 1..23: mol_type = other RNA
gtaacagtcggaggcgcgacggc

SEQ ID NO: 523 - RNA, 21 nt, synthetic construct
  source 1..21: mol_type = other RNA
gtcgcgcctccgactgttacc

SEQ ID NO: 524 - RNA, 23 nt, synthetic construct
  source 1..23: mol_type = other RNA
ggtaacagtcggaggcgcgacgg

SEQ ID NO: 525 - RNA, 21 nt, synthetic construct
  source 1..21: mol_type = other RNA
tcgcgcctccgactgttaccc

SEQ ID NO: 526 - RNA, 23 nt, synthetic construct
  source 1..23: mol_type = other RNA
gggtaacagtcggaggcgcgacg

SEQ ID NO: 527 - RNA, 21 nt, synthetic construct
  source 1..21: mol_type = other RNA
cgcgcctccgactgttacccc

SEQ ID NO: 528 - RNA, 23 nt, synthetic construct
  source 1..23: mol_type = other RNA
ggggtaacagtcggaggcgcgac

SEQ ID NO: 529 - RNA, 21 nt, synthetic construct
  source 1..21: mol_type = other RNA
ccttccgaacaagcaccgact

SEQ ID NO: 530 - RNA, 23 nt, synthetic construct
  source 1..23: mol_type = other RNA
agtcggtgcttgttcggaaggag

SEQ ID NO: 531 - RNA, 21 nt, synthetic construct
  source 1..21: mol_type = other RNA
agttatcgaggcacatactcc

SEQ ID NO: 532 - RNA, 23 nt, synthetic construct
  source 1..23: mol_type = other RNA
ggagtatgtgcctcgataactct

SEQ ID NO: 533 - RNA, 21 nt, synthetic construct
  source 1..21: mol_type = other RNA
acaccacactcgcatagtcgg

SEQ ID NO: 534 - RNA, 23 nt, synthetic construct
  source 1..23: mol_type = other RNA
ccgactatgcgagtgtggtgtca

SEQ ID NO: 535 - RNA, 21 nt, synthetic construct
  source 1..21: mol_type = other RNA
caccacactcgcatagtcgga

SEQ ID NO: 536 - RNA, 23 nt, synthetic construct
  source 1..23: mol_type = other RNA
tccgactatgcgagtgtggtgtc

SEQ ID NO: 537 - RNA, 21 nt, synthetic construct
  source 1..21: mol_type = other RNA
accacactcgcatagtcggac

SEQ ID NO: 538 - RNA, 23 nt, synthetic construct
  source 1..23: mol_type = other RNA
gtccgactatgcgagtgtggtgt

SEQ ID NO: 539 - RNA, 21 nt, synthetic construct
  source 1..21: mol_type = other RNA
ccacactcgcatagtcggacc

SEQ ID NO: 540 - RNA, 23 nt, synthetic construct
  source 1..23: mol_type = other RNA
ggtccgactatgcgagtgtggtg

SEQ ID NO: 541 - RNA, 21 nt, synthetic construct
  source 1..21: mol_type = other RNA
cacactcgcatagtcggaccc

SEQ ID NO: 542 - RNA, 23 nt, synthetic construct
  source 1..23: mol_type = other RNA
gggtccgactatgcgagtgtggt

SEQ ID NO: 543 - RNA, 21 nt, synthetic construct
  source 1..21: mol_type = other RNA
acactcgcatagtcggacccc

SEQ ID NO: 544 - RNA, 23 nt, synthetic construct
  source 1..23: mol_type = other RNA
ggggtccgactatgcgagtgtgg

SEQ ID NO: 545 - RNA, 21 nt, synthetic construct
  source 1..21: mol_type = other RNA
cactcgcatagtcggacccca

SEQ ID NO: 546 - RNA, 23 nt, synthetic construct
  source 1..23: mol_type = other RNA
tggggtccgactatgcgagtgtg

SEQ ID NO: 547 - RNA, 21 nt, synthetic construct
  source 1..21: mol_type = other RNA
actcgcatagtcggaccccag

SEQ ID NO: 548 - RNA, 23 nt, synthetic construct
  source 1..23: mol_type = other RNA
ctggggtccgactatgcgagtgt

SEQ ID NO: 549 - RNA, 21 nt, synthetic construct
  source 1..21: mol_type = other RNA
ctcgcatagtcggaccccaga

SEQ ID NO: 550 - RNA, 23 nt, synthetic construct
  source 1..23: mol_type = other RNA
tctggggtccgactatgcgagtg

SEQ ID NO: 551 - RNA, 21 nt, synthetic construct
  source 1..21: mol_type = other RNA
tcgcatagtcggaccccagaa

SEQ ID NO: 552 - RNA, 23 nt, synthetic construct
  source 1..23: mol_type = other RNA
ttctggggtccgactatgcgagt

SEQ ID NO: 553 - RNA, 21 nt, synthetic construct
  source 1..21: mol_type = other RNA
catagtcggaccccagaatac

SEQ ID NO: 554 - RNA, 23 nt, synthetic construct
  source 1..23: mol_type = other RNA
gtattctggggtccgactatgcg

SEQ ID NO: 555 - RNA, 21 nt, synthetic construct
  source 1..21: mol_type = other RNA
agccccttattgttatacgag

SEQ ID NO: 556 - RNA, 23 nt, synthetic construct
  source 1..23: mol_type = other RNA
ctcgtataacaataaggggctgc

SEQ ID NO: 557 - RNA, 21 nt, synthetic construct
  source 1..21: mol_type = other RNA
attgttatacgagggatccca

SEQ ID NO: 558 - RNA, 23 nt, synthetic construct
  source 1..23: mol_type = other RNA
tgggatccctcgtataacaataa

SEQ ID NO: 559 - RNA, 21 nt, synthetic construct
  source 1..21: mol_type = other RNA
actgccgtcgcgcctccaact

SEQ ID NO: 560 - RNA, 23 nt, synthetic construct
  source 1..23: mol_type = other RNA
agttggaggcgcgacggcagtcc

SEQ ID NO: 561 - RNA, 21 nt, synthetic construct
  source 1..21: mol_type = other RNA
ctgccgtcgcgcctccaacta

SEQ ID NO: 562 - RNA, 23 nt, synthetic construct
  source 1..23: mol_type = other RNA
tagttggaggcgcgacggcagtc

SEQ ID NO: 563 - RNA, 21 nt, synthetic construct
  source 1..21: mol_type = other RNA
tgccgtcgcgcctccaactat

SEQ ID NO: 564 - RNA, 23 nt, synthetic construct
  source 1..23: mol_type = other RNA
atagttggaggcgcgacggcagt

SEQ ID NO: 565 - RNA, 21 nt, synthetic construct
  source 1..21: mol_type = other RNA
gtcgcgcctccaactattacc

SEQ ID NO: 566 - RNA, 23 nt, synthetic construct
  source 1..23: mol_type = other RNA
ggtaatagttggaggcgcgacgg

SEQ ID NO: 567 - RNA, 21 nt, synthetic construct
  source 1..21: mol_type = other RNA
gcctccaactattaccccgat

SEQ ID NO: 568 - RNA, 23 nt, synthetic construct
  source 1..23: mol_type = other RNA
atcggggtaatagttggaggcgc

SEQ ID NO: 569 - RNA, 21 nt, synthetic construct
  source 1..21: mol_type = other RNA
ggagtgctaccacggaaatgg

SEQ ID NO: 570 - RNA, 23 nt, synthetic construct
  source 1..23: mol_type = other RNA
ccatttccgtggtagcactcctg

SEQ ID NO: 571 - RNA, 21 nt, synthetic construct
  source 1..21: mol_type = other RNA
gagtgctaccacggaaatgga

SEQ ID NO: 572 - RNA, 23 nt, synthetic construct
  source 1..23: mol_type = other RNA
tccatttccgtggtagcactcct

SEQ ID NO: 573 - RNA, 21 nt, synthetic construct
  source 1..21: mol_type = other RNA
agtgctaccacggaaatggac

SEQ ID NO: 574 - RNA, 23 nt, synthetic construct
  source 1..23: mol_type = other RNA
gtccatttccgtggtagcactcc

SEQ ID NO: 575 - RNA, 21 nt, synthetic construct
  source 1..21: mol_type = other RNA
tcaaggcacatacttcattac

SEQ ID NO: 576 - RNA, 23 nt, synthetic construct
  source 1..23: mol_type = other RNA
gtaatgaagtatgtgccttgata

SEQ ID NO: 577 - RNA, 21 nt, synthetic construct
  source 1..21: mol_type = other RNA
ggcacatacttcattactgtc

SEQ ID NO: 578 - RNA, 23 nt, synthetic construct
  source 1..23: mol_type = other RNA
gacagtaatgaagtatgtgcctt

SEQ ID NO: 579 - RNA, 21 nt, synthetic construct
  source 1..21: mol_type = other RNA
cattactgtcacaggaagaac

SEQ ID NO: 580 - RNA, 23 nt, synthetic construct
  source 1..23: mol_type = other RNA
gttcttcctgtgacagtaatgaa

SEQ ID NO: 581 - RNA, 21 nt, synthetic construct
  source 1..21: mol_type = other RNA
cttggtgttatacaacagatc

SEQ ID NO: 582 - RNA, 23 nt, synthetic construct
  source 1..23: mol_type = other RNA
gatctgttgtataacaccaaggg

SEQ ID NO: 583 - RNA, 21 nt, synthetic construct
  source 1..21: mol_type = other RNA
aacagatcccagtgtcaggtg

SEQ ID NO: 584 - RNA, 23 nt, synthetic construct
  source 1..23: mol_type = other RNA
cacctgacactgggatctgttgt

SEQ ID NO: 585 - RNA, 21 nt, synthetic construct
  source 1..21: mol_type = other RNA
acctgacacgatgctcagatg

SEQ ID NO: 586 - RNA, 23 nt, synthetic construct
  source 1..23: mol_type = other RNA
catctgagcatcgtgtcaggttg

SEQ ID NO: 587 - RNA, 21 nt, synthetic construct
  source 1..21: mol_type = other RNA
gcagaatggactgccttcgtc

SEQ ID NO: 588 - RNA, 23 nt, synthetic construct
  source 1..23: mol_type = other RNA
gacgaaggcagtccattctgcat

SEQ ID NO: 589 - RNA, 21 nt, synthetic construct
  source 1..21: mol_type = other RNA
tcgtccctccgaatgttattc

SEQ ID NO: 590 - RNA, 23 nt, synthetic construct
  source 1..23: mol_type = other RNA
gaataacattcggagggacgaag

SEQ ID NO: 591 - RNA, 21 nt, synthetic construct
  source 1..21: mol_type = other RNA
cgtccctccgaatgttattct

SEQ ID NO: 592 - RNA, 23 nt, synthetic construct
  source 1..23: mol_type = other RNA
agaataacattcggagggacgaa

SEQ ID NO: 593 - RNA, 21 nt, synthetic construct
  source 1..21: mol_type = other RNA
gtccctccgaatgttattctg

SEQ ID NO: 594 - RNA, 23 nt, synthetic construct
  source 1..23: mol_type = other RNA
cagaataacattcggagggacga

SEQ ID NO: 595 - RNA, 21 nt, synthetic construct
  source 1..21: mol_type = other RNA
cctccgaatgttattctggct

SEQ ID NO: 596 - RNA, 23 nt, synthetic construct
  source 1..23: mol_type = other RNA
agccagaataacattcggaggga

SEQ ID NO: 597 - RNA, 21 nt, synthetic construct
  source 1..21: mol_type = other RNA
tattctggctccaagcctaga

SEQ ID NO: 598 - RNA, 23 nt, synthetic construct
  source 1..23: mol_type = other RNA
tctaggcttggagccagaataac

SEQ ID NO: 599 - RNA, 21 nt, synthetic construct
  source 1..21: mol_type = other RNA
taccattatggacagagttac

SEQ ID NO: 600 - RNA, 23 nt, synthetic construct
  source 1..23: mol_type = other RNA
gtaactctgtccataatggtagt

SEQ ID NO: 601 - RNA, 21 nt, synthetic construct
  source 1..21: mol_type = other RNA
accattatggacagagttacc

SEQ ID NO: 602 - RNA, 23 nt, synthetic construct
  source 1..23: mol_type = other RNA
ggtaactctgtccataatggtag

SEQ ID NO: 603 - RNA, 21 nt, synthetic construct
  source 1..21: mol_type = other RNA
accagcatagtcggaccccag

SEQ ID NO: 604 - RNA, 23 nt, synthetic construct
  source 1..23: mol_type = other RNA
ctggggtccgactatgctggtgt

SEQ ID NO: 605 - RNA, 21 nt, synthetic construct
  source 1..21: mol_type = other RNA
ccagcatagtcggaccccaga

SEQ ID NO: 606 - RNA, 23 nt, synthetic construct
  source 1..23: mol_type = other RNA
tctggggtccgactatgctggtg

SEQ ID NO: 607 - RNA, 21 nt, synthetic construct
  source 1..21: mol_type = other RNA
gtccttgcaactctcacggtg

SEQ ID NO: 608 - RNA, 23 nt, synthetic construct
  source 1..23: mol_type = other RNA
caccgtgagagttgcaaggacac

SEQ ID NO: 609 - RNA, 21 nt, synthetic construct
  source 1..21: mol_type = other RNA
gagttatcgaggctcattctc

SEQ ID NO: 610 - RNA, 23 nt, synthetic construct
  source 1..23: mol_type = other RNA
gagaatgagcctcgataactctg

SEQ ID NO: 611 - RNA, 21 nt, synthetic construct
  source 1..21: mol_type = other RNA
agttatcgaggctcattctct

SEQ ID NO: 612 - RNA, 23 nt, synthetic construct
  source 1..23: mol_type = other RNA
agagaatgagcctcgataactct

SEQ ID NO: 613 - RNA, 21 nt, synthetic construct
  source 1..21: mol_type = other RNA
agaggacaacagaatattatc

SEQ ID NO: 614 - RNA, 23 nt, synthetic construct
  source 1..23: mol_type = other RNA
gataatattctgttgtcctctga

SEQ ID NO: 615 - RNA, 21 nt, synthetic construct
  source 1..21: mol_type = other RNA
atgctgagattagtccttggt

SEQ ID NO: 616 - RNA, 23 nt, synthetic construct
  source 1..23: mol_type = other RNA
accaaggactaatctcagcatct

SEQ ID NO: 617 - RNA, 21 nt, synthetic construct
  source 1..21: mol_type = other RNA
agattagtccttggtgttata

SEQ ID NO: 618 - RNA, 23 nt, synthetic construct
  source 1..23: mol_type = other RNA
tataacaccaaggactaatctca

SEQ ID NO: 619 - RNA, 21 nt, synthetic construct
  source 1..21: mol_type = other RNA
attagtccttggtgttatacc

SEQ ID NO: 620 - RNA, 23 nt, synthetic construct
  source 1..23: mol_type = other RNA
ggtataacaccaaggactaatct

SEQ ID NO: 621 - RNA, 21 nt, synthetic construct
  source 1..21: mol_type = other RNA
ccaatgtcagatgggagtact

SEQ ID NO: 622 - RNA, 23 nt, synthetic construct
  source 1..23: mol_type = other RNA
agtactcccatctgacattggga

SEQ ID NO: 623 - RNA, 21 nt, synthetic construct
  source 1..21: mol_type = other RNA
atcaagtgtccttgcgacgtc

SEQ ID NO: 624 - RNA, 23 nt, synthetic construct
  source 1..23: mol_type = other RNA
gacgtcgcaaggacacttgattc

SEQ ID NO: 625 - RNA, 21 nt, synthetic construct
  source 1..21: mol_type = other RNA
caagtgtccttgcgacgtcca

SEQ ID NO: 626 - RNA, 23 nt, synthetic construct
  source 1..23: mol_type = other RNA
tggacgtcgcaaggacacttgat

SEQ ID NO: 627 - RNA, 21 nt, synthetic construct
  source 1..21: mol_type = other RNA
tgtccttgcgacgtccacggc

SEQ ID NO: 628 - RNA, 23 nt, synthetic construct
  source 1..23: mol_type = other RNA
gccgtggacgtcgcaaggacact

SEQ ID NO: 629 - RNA, 21 nt, synthetic construct
  source 1..21: mol_type = other RNA
gtccttgcgacgtccacggct

SEQ ID NO: 630 - RNA, 23 nt, synthetic construct
  source 1..23: mol_type = other RNA
agccgtggacgtcgcaaggacac

SEQ ID NO: 631 - RNA, 21 nt, synthetic construct
  source 1..21: mol_type = other RNA
tgcgacgtccacggctgtttc

SEQ ID NO: 632 - RNA, 23 nt, synthetic construct
  source 1..23: mol_type = other RNA
gaaacagccgtggacgtcgcaag

SEQ ID NO: 633 - RNA, 21 nt, synthetic construct
  source 1..21: mol_type = other RNA
ctgtttctgaacaagcaccaa

SEQ ID NO: 634 - RNA, 23 nt, synthetic construct
  source 1..23: mol_type = other RNA
ttggtgcttgttcagaaacagcc

SEQ ID NO: 635 - RNA, 21 nt, synthetic construct
  source 1..21: mol_type = other RNA
cacagtccaggactgctacca

SEQ ID NO: 636 - RNA, 23 nt, synthetic construct
  source 1..23: mol_type = other RNA
tggtagcagtcctggactgtggg

SEQ ID NO: 637 - RNA, 21 nt, synthetic construct
  source 1..21: mol_type = other RNA
agttatcgaggctcattctcc

SEQ ID NO: 638 - RNA, 23 nt, synthetic construct
  source 1..23: mol_type = other RNA
ggagaatgagcctcgataactct

SEQ ID NO: 639 - RNA, 21 nt, synthetic construct
  source 1..21: mol_type = other RNA
agattcgcccttggtgttata

SEQ ID NO: 640 - RNA, 23 nt, synthetic construct
  source 1..23: mol_type = other RNA
tataacaccaagggcgaatctca

SEQ ID NO: 641 - RNA, 21 nt, synthetic construct
  source 1..21: mol_type = other RNA
gaatcaactctcctcacaact

SEQ ID NO: 642 - RNA, 23 nt, synthetic construct
  source 1..23: mol_type = other RNA
agttgtgaggagagttgattcca

SEQ ID NO: 643 - RNA, 21 nt, synthetic construct
  source 1..21: mol_type = other RNA
tctcctcacaactcccacggt

SEQ ID NO: 644 - RNA, 23 nt, synthetic construct
  source 1..23: mol_type = other RNA
accgtgggagttgtgaggagagt

SEQ ID NO: 645 - RNA, 21 nt, synthetic construct
  source 1..21: mol_type = other RNA
ctcacaactcccacggtggtc

SEQ ID NO: 646 - RNA, 23 nt, synthetic construct
  source 1..23: mol_type = other RNA
gaccaccgtgggagttgtgagga

SEQ ID NO: 647 - RNA, 21 nt, synthetic construct
  source 1..21: mol_type = other RNA
ctcccacggtggtcccagttc

SEQ ID NO: 648 - RNA, 23 nt, synthetic construct
  source 1..23: mol_type = other RNA
gaactgggaccaccgtgggagtt

SEQ ID NO: 649 - RNA, 21 nt, synthetic construct
  source 1..21: mol_type = other RNA
ctggggtccaggactgctacc

SEQ ID NO: 650 - RNA, 23 nt, synthetic construct
  source 1..23: mol_type = other RNA
ggtagcagtcctggaccccagtg

SEQ ID NO: 651 - RNA, 21 nt, synthetic construct
  source 1..21: mol_type = other RNA
ccgaggtgatggacagagtta

SEQ ID NO: 652 - RNA, 23 nt, synthetic construct
  source 1..23: mol_type = other RNA
taactctgtccatcacctcggta

SEQ ID NO: 653 - RNA, 21 nt, synthetic construct
  source 1..21: mol_type = other RNA
acagagttatcgaggcacact

SEQ ID NO: 654 - RNA, 23 nt, synthetic construct
  source 1..23: mol_type = other RNA
agtgtgcctcgataactctgtcc

SEQ ID NO: 655 - RNA, 21 nt, synthetic construct
  source 1..21: mol_type = other RNA
cagagttatcgaggcacactc

SEQ ID NO: 656 - RNA, 23 nt, synthetic construct
  source 1..23: mol_type = other RNA
gagtgtgcctcgataactctgtc

SEQ ID NO: 657 - RNA, 21 nt, synthetic construct
  source 1..21: mol_type = other RNA
cagtcttggtcgtctatgaca

SEQ ID NO: 658 - RNA, 23 nt, synthetic construct
  source 1..23: mol_type = other RNA
tgtcatagacgaccaagactgac

SEQ ID NO: 659 - RNA, 21 nt, synthetic construct
  source 1..21: mol_type = other RNA
cgtctatgacaccacattggc

SEQ ID NO: 660 - RNA, 23 nt, synthetic construct
  source 1..23: mol_type = other RNA
gccaatgtggtgtcatagacgac

SEQ ID NO: 661 - RNA, 21 nt, synthetic construct
  source 1..21: mol_type = other RNA
atgacaccacattggcatcgg

SEQ ID NO: 662 - RNA, 23 nt, synthetic construct
  source 1..23: mol_type = other RNA
ccgatgccaatgtggtgtcatag

SEQ ID NO: 663 - RNA, 21 nt, synthetic construct
  source 1..21: mol_type = other RNA
ccacattggcatcggaggatc

SEQ ID NO: 664 - RNA, 23 nt, synthetic construct
  source 1..23: mol_type = other RNA
gatcctccgatgccaatgtggtg

SEQ ID NO: 665 - RNA, 21 nt, synthetic construct
  source 1..21: mol_type = other RNA
catcggaggatcccattatac

SEQ ID NO: 666 - RNA, 23 nt, synthetic construct
  source 1..23: mol_type = other RNA
gtataatgggatcctccgatgcc

SEQ ID NO: 667 - RNA, 21 nt, synthetic construct
  source 1..21: mol_type = other RNA
atcggaggatcccattatact

SEQ ID NO: 668 - RNA, 23 nt, synthetic construct
  source 1..23: mol_type = other RNA
agtataatgggatcctccgatgc

SEQ ID NO: 669 - RNA, 21 nt, synthetic construct
  source 1..21: mol_type = other RNA
ggaggatcccattatactatc

SEQ ID NO: 670 - RNA, 23 nt, synthetic construct
  source 1..23: mol_type = other RNA
gatagtataatgggatcctccga

SEQ ID NO: 671 - RNA, 21 nt, synthetic construct
  source 1..21: mol_type = other RNA
gaggatcccattatactatcc

SEQ ID NO: 672 - RNA, 23 nt, synthetic construct
  source 1..23: mol_type = other RNA
ggatagtataatgggatcctccg

SEQ ID NO: 673 - RNA, 21 nt, synthetic construct
  source 1..21: mol_type = other RNA
tactgcaacctgacacgatgt

SEQ ID NO: 674 - RNA, 23 nt, synthetic construct
  source 1..23: mol_type = other RNA
acatcgtgtcaggttgcagtact

SEQ ID NO: 675 - RNA, 21 nt, synthetic construct
  source 1..21: mol_type = other RNA
actgcaacctgacacgatgtc

SEQ ID NO: 676 - RNA, 23 nt, synthetic construct
  source 1..23: mol_type = other RNA
gacatcgtgtcaggttgcagtac

SEQ ID NO: 677 - RNA, 21 nt, synthetic construct
  source 1..21: mol_type = other RNA
cagtgacagaatcgagtgtcc

SEQ ID NO: 678 - RNA, 23 nt, synthetic construct
  source 1..23: mol_type = other RNA
ggacactcgattctgtcactgga

SEQ ID NO: 679 - RNA, 21 nt, synthetic construct
  source 1..21: mol_type = other RNA
gacagaatcgagtgtcctcac

SEQ ID NO: 680 - RNA, 23 nt, synthetic construct
  source 1..23: mol_type = other RNA
gtgaggacactcgattctgtcac

SEQ ID NO: 681 - RNA, 21 nt, synthetic construct
  source 1..21: mol_type = other RNA
acggagttatcgaggcatatc

SEQ ID NO: 682 - RNA, 23 nt, synthetic construct
  source 1..23: mol_type = other RNA
gatatgcctcgataactccgtcc

SEQ ID NO: 683 - RNA, 21 nt, synthetic construct
  source 1..21: mol_type = other RNA
cggagttatcgaggcatatcc

SEQ ID NO: 684 - RNA, 23 nt, synthetic construct
  source 1..23: mol_type = other RNA
ggatatgcctcgataactccgtc

SEQ ID NO: 685 - RNA, 21 nt, synthetic construct
  source 1..21: mol_type = other RNA
ggagttatcgaggcatatcct

SEQ ID NO: 686 - RNA, 23 nt, synthetic construct
  source 1..23: mol_type = other RNA
aggatatgcctcgataactccgt

SEQ ID NO: 687 - RNA, 21 nt, synthetic construct
  source 1..21: mol_type = other RNA
gagttatcgaggcatatcctc

SEQ ID NO: 688 - RNA, 23 nt, synthetic construct
  source 1..23: mol_type = other RNA
gaggatatgcctcgataactccg

SEQ ID NO: 689 - RNA, 21 nt, synthetic construct
  source 1..21: mol_type = other RNA
catatcctccaccactgtcac

SEQ ID NO: 690 - RNA, 23 nt, synthetic construct
  source 1..23: mol_type = other RNA
gtgacagtggtggaggatatgcc

SEQ ID NO: 691 - RNA, 21 nt, synthetic construct
  source 1..21: mol_type = other RNA
aatcttggtcatctatgatac

SEQ ID NO: 692 - RNA, 23 nt, synthetic construct
  source 1..23: mol_type = other RNA
gtatcatagatgaccaagattga

SEQ ID NO: 693 - RNA, 21 nt, synthetic construct
  source 1..21: mol_type = other RNA
ccgagaactactgcaggaatc

SEQ ID NO: 694 - RNA, 23 nt, synthetic construct
  source 1..23: mol_type = other RNA
gattcctgcagtagttctcggtc

SEQ ID NO: 695 - RNA, 21 nt, synthetic construct
  source 1..21: mol_type = other RNA
ccctggtgttacacaaccgat

SEQ ID NO: 696 - RNA, 23 nt, synthetic construct
  source 1..23: mol_type = other RNA
atcggttgtgtaacaccagggtt

SEQ ID NO: 697 - RNA, 21 nt, synthetic construct
  source 1..21: mol_type = other RNA
cctggtgttacacaaccgatc

SEQ ID NO: 698 - RNA, 23 nt, synthetic construct
  source 1..23: mol_type = other RNA
gatcggttgtgtaacaccagggt

SEQ ID NO: 699 - RNA, 21 nt, synthetic construct
  source 1..21: mol_type = other RNA
ctggtgttacacaaccgatcc

SEQ ID NO: 700 - RNA, 23 nt, synthetic construct
  source 1..23: mol_type = other RNA
ggatcggttgtgtaacaccaggg

SEQ ID NO: 701 - RNA, 21 nt, synthetic construct
  source 1..21: mol_type = other RNA
ccgtgtgtgaggtgggagtac

SEQ ID NO: 702 - RNA, 23 nt, synthetic construct
  source 1..23: mol_type = other RNA
gtactcccacctcacacacggat

SEQ ID NO: 703 - RNA, 21 nt, synthetic construct
  source 1..21: mol_type = other RNA
cagtgctaccatggtaatggc

SEQ ID NO: 704 - RNA, 23 nt, synthetic construct
  source 1..23: mol_type = other RNA
gccattaccatggtagcactgcc

SEQ ID NO: 705 - RNA, 21 nt, synthetic construct
  source 1..21: mol_type = other RNA
agtgctaccatggtaatggcc

SEQ ID NO: 706 - RNA, 23 nt, synthetic construct
  source 1..23: mol_type = other RNA
ggccattaccatggtagcactgc

SEQ ID NO: 707 - RNA, 21 nt, synthetic construct
  source 1..21: mol_type = other RNA
ccagagttatcgaggcacatt

SEQ ID NO: 708 - RNA, 23 nt, synthetic construct
  source 1..23: mol_type = other RNA
aatgtgcctcgataactctggcc

SEQ ID NO: 709 - RNA, 21 nt, synthetic construct
  source 1..21: mol_type = other RNA
cagagttatcgaggcacattc

SEQ ID NO: 710 - RNA, 23 nt, synthetic construct
  source 1..23: mol_type = other RNA
gaatgtgcctcgataactctggc

SEQ ID NO: 711 - RNA, 21 nt, synthetic construct
  source 1..21: mol_type = other RNA
agatgccgatacaggcccttg

SEQ ID NO: 712 - RNA, 23 nt, synthetic construct
  source 1..23: mol_type = other RNA
caagggcctgtatcggcatctgg

SEQ ID NO: 713 - RNA, 21 nt, synthetic construct
  source 1..21: mol_type = other RNA
agcatcaggtgggagtactgc

SEQ ID NO: 714 - RNA, 23 nt, synthetic construct
  source 1..23: mol_type = other RNA
gcagtactcccacctgatgctgg

SEQ ID NO: 715 - RNA, 21 nt, synthetic construct
  source 1..21: mol_type = other RNA
acctgacgcgatgctcagaca

SEQ ID NO: 716 - RNA, 23 nt, synthetic construct
  source 1..23: mol_type = other RNA
tgtctgagcatcgcgtcaggttg

SEQ ID NO: 717 - RNA, 21 nt, synthetic construct
  source 1..21: mol_type = other RNA
tgtggtcgctcctccgactgt

SEQ ID NO: 718 - RNA, 23 nt, synthetic construct
  source 1..23: mol_type = other RNA
acagtcggaggagcgaccacagt

SEQ ID NO: 719 - RNA, 21 nt, synthetic construct
  source 1..21: mol_type = other RNA
tagacacagcacgttcattcc

SEQ ID NO: 720 - RNA, 23 nt, synthetic construct
  source 1..23: mol_type = other RNA
ggaatgaacgtgctgtgtctatg

SEQ ID NO: 721 - RNA, 21 nt, synthetic construct
  source 1..21: mol_type = other RNA
agacacagcacgttcattcca

SEQ ID NO: 722 - RNA, 23 nt, synthetic construct
  source 1..23: mol_type = other RNA
tggaatgaacgtgctgtgtctat

SEQ ID NO: 723 - RNA, 21 nt, synthetic construct
  source 1..21: mol_type = other RNA
ctttttgactactgtgatatc

SEQ ID NO: 724 - RNA, 23 nt, synthetic construct
  source 1..23: mol_type = other RNA
gatatcacagtagtcaaaaagtt

SEQ ID NO: 725 - RNA, 21 nt, synthetic construct
  source 1..21: mol_type = other RNA
tttttgactactgtgatatcc

SEQ ID NO: 726 - RNA, 23 nt, synthetic construct
  source 1..23: mol_type = other RNA
ggatatcacagtagtcaaaaagt

SEQ ID NO: 727 - RNA, 21 nt, synthetic construct
  source 1..21: mol_type = other RNA
ttttgactactgtgatatccc

SEQ ID NO: 728 - RNA, 23 nt, synthetic construct
  source 1..23: mol_type = other RNA
gggatatcacagtagtcaaaaag

SEQ ID NO: 729 - RNA, 21 nt, synthetic construct
  source 1..21: mol_type = other RNA
ctgtggaggcaccttaatatc

SEQ ID NO: 730 - RNA, 23 nt, synthetic construct
  source 1..23: mol_type = other RNA
gatattaaggtgcctccacagaa

SEQ ID NO: 731 - RNA, 21 nt, synthetic construct
  source 1..21: mol_type = other RNA
tgtggaggcaccttaatatcc

SEQ ID NO: 732 - RNA, 23 nt, synthetic construct
  source 1..23: mol_type = other RNA
ggatattaaggtgcctccacaga

SEQ ID NO: 733 - RNA, 21 nt, synthetic construct
  source 1..21: mol_type = other RNA
aagtgaacctcgaatctcatg

SEQ ID NO: 734 - RNA, 23 nt, synthetic construct
  source 1..23: mol_type = other RNA
catgagattcgaggttcacttct

SEQ ID NO: 735 - RNA, 21 nt, synthetic construct
  source 1..21: mol_type = other RNA
agtgaacctcgaatctcatgt

SEQ ID NO: 736 - RNA, 23 nt, synthetic construct
  source 1..23: mol_type = other RNA
acatgagattcgaggttcacttc

SEQ ID NO: 737 - RNA, 21 nt, synthetic construct
  source 1..21: mol_type = other RNA
cccacacaagcagatattgcc

SEQ ID NO: 738 - RNA, 23 nt, synthetic construct
  source 1..23: mol_type = other RNA
ggcaatatctgcttgtgtgggct

SEQ ID NO: 739 - RNA, 21 nt, synthetic construct
  source 1..21: mol_type = other RNA
tcatcactgacaaagtaatgc

SEQ ID NO: 740 - RNA, 23 nt, synthetic construct
  source 1..23: mol_type = other RNA
gcattactttgtcagtgatgacg

SEQ ID NO: 741 - RNA, 21 nt, synthetic construct
  source 1..21: mol_type = other RNA
catcactgacaaagtaatgcc

SEQ ID NO: 742 - RNA, 23 nt, synthetic construct
  source 1..23: mol_type = other RNA
ggcattactttgtcagtgatgac

SEQ ID NO: 743 - RNA, 21 nt, synthetic construct
  source 1..21: mol_type = other RNA
aagcccagctccttgttattg

SEQ ID NO: 744 - RNA, 23 nt, synthetic construct
  source 1..23: mol_type = other RNA
caataacaaggagctgggcttcc

SEQ ID NO: 745 - RNA, 21 nt, synthetic construct
  source 1..21: mol_type = other RNA
cccagctccttgttattgaga

SEQ ID NO: 746 - RNA, 23 nt, synthetic construct
  source 1..23: mol_type = other RNA
tctcaataacaaggagctgggct

SEQ ID NO: 747 - RNA, 21 nt, synthetic construct
  source 1..21: mol_type = other RNA
ttgagaatgaagtgtgcaatc

SEQ ID NO: 748 - RNA, 23 nt, synthetic construct
  source 1..23: mol_type = other RNA
gattgcacacttcattctcaata

SEQ ID NO: 749 - RNA, 21 nt, synthetic construct
  source 1..21: mol_type = other RNA
gaagtgtgcaatcactataag

SEQ ID NO: 750 - RNA, 23 nt, synthetic construct
  source 1..23: mol_type = other RNA
cttatagtgattgcacacttcat

SEQ ID NO: 751 - RNA, 21 nt, synthetic construct
  source 1..21: mol_type = other RNA
aagtgtgcaatcactataagt

SEQ ID NO: 752 - RNA, 23 nt, synthetic construct
  source 1..23: mol_type = other RNA
acttatagtgattgcacacttca

SEQ ID NO: 753 - RNA, 21 nt, synthetic construct
  source 1..21: mol_type = other RNA
cactataagtatatttgtgct

SEQ ID NO: 754 - RNA, 23 nt, synthetic construct
  source 1..23: mol_type = other RNA
agcacaaatatacttatagtgat

SEQ ID NO: 755 - RNA, 21 nt, synthetic construct
  source 1..21: mol_type = other RNA
agtatatttgtgctgagcatt

SEQ ID NO: 756 - RNA, 23 nt, synthetic construct
  source 1..23: mol_type = other RNA
aatgctcagcacaaatatactta

SEQ ID NO: 757 - RNA, 21 nt, synthetic construct
  source 1..21: mol_type = other RNA
gtctatgctcgtgtttcaagg

SEQ ID NO: 758 - RNA, 23 nt, synthetic construct
  source 1..23: mol_type = other RNA
ccttgaaacacgagcatagacac

SEQ ID NO: 759 - RNA, 21 nt, synthetic construct
  source 1..21: mol_type = other RNA
acttggattgagggaatgatg

SEQ ID NO: 760 - RNA, 23 nt, synthetic construct
  source 1..23: mol_type = other RNA
catcattccctcaatccaagtaa

SEQ ID NO: 761 - RNA, 21 nt, synthetic construct
  source 1..21: mol_type = other RNA
catcaacctacttagaagctg

SEQ ID NO: 762 - RNA, 23 nt, synthetic construct
  source 1..23: mol_type = other RNA
cagcttctaagtaggttgatgct

SEQ ID NO: 763 - RNA, 21 nt, synthetic construct
  source 1..21: mol_type = other RNA
cctacttagaagctgaaacgt

SEQ ID NO: 764 - RNA, 23 nt, synthetic construct
  source 1..23: mol_type = other RNA
acgtttcagcttctaagtaggtt

SEQ ID NO: 765 - RNA, 21 nt, synthetic construct
  source 1..21: mol_type = other RNA
aataatagacagcaatcaaac

SEQ ID NO: 766 - RNA, 23 nt, synthetic construct
  source 1..23: mol_type = other RNA
gtttgattgctgtctattatttc

SEQ ID NO: 767 - RNA, 21 nt, synthetic construct
  source 1..21: mol_type = other RNA
tagacagcaatcaaacgaaga

SEQ ID NO: 768 - RNA, 23 nt, synthetic construct
  source 1..23: mol_type = other RNA
tcttcgtttgattgctgtctatt

SEQ ID NO: 769 - RNA, 21 nt, synthetic construct
  source 1..21: mol_type = other RNA
ttttgtgtataagcttttaag

SEQ ID NO: 770 - RNA, 23 nt, synthetic construct
  source 1..23: mol_type = other RNA
cttaaaagcttatacacaaaaat

SEQ ID NO: 771 - RNA, 21 nt, synthetic construct
  source 1..21: mol_type = other RNA
ttgtgtataagcttttaaggt

SEQ ID NO: 772 - RNA, 23 nt, synthetic construct
  source 1..23: mol_type = other RNA
accttaaaagcttatacacaaaa

SEQ ID NO: 773 - RNA, 21 nt, synthetic construct
  source 1..21: mol_type = other RNA
tgtgtataagcttttaaggtc

SEQ ID NO: 774 - RNA, 23 nt, synthetic construct
  source 1..23: mol_type = other RNA
gaccttaaaagcttatacacaaa

SEQ ID NO: 775 - RNA, 21 nt, synthetic construct
  source 1..21: mol_type = other RNA
taaggtctgactgacaaattc

SEQ ID NO: 776 - RNA, 23 nt, synthetic construct
  source 1..23: mol_type = other RNA
gaatttgtcagtcagaccttaaa

SEQ ID NO: 777 - RNA, 21 nt, synthetic construct
  source 1..21: mol_type = other RNA
ctgacaaattctgtattaagg

SEQ ID NO: 778 - RNA, 23 nt, synthetic construct
  source 1..23: mol_type = other RNA
ccttaatacagaatttgtcagtc

SEQ ID NO: 779 - RNA, 21 nt, synthetic construct
  source 1..21: mol_type = other RNA
tgacaaattctgtattaaggt

SEQ ID NO: 780 - RNA, 23 nt, synthetic construct
  source 1..23: mol_type = other RNA
accttaatacagaatttgtcagt

SEQ ID NO: 781 - RNA, 21 nt, synthetic construct
  source 1..21: mol_type = other RNA
tatgacatttgttaaaaataa

SEQ ID NO: 782 - RNA, 23 nt, synthetic construct
  source 1..23: mol_type = other RNA
ttatttttaacaaatgtcatagc

SEQ ID NO: 783 - RNA, 21 nt, synthetic construct
  source 1..21: mol_type = other RNA
ataaactctgcacttattttg

SEQ ID NO: 784 - RNA, 23 nt, synthetic construct
  source 1..23: mol_type = other RNA
caaaataagtgcagagtttattt

SEQ ID NO: 785 - RNA, 20 nt, synthetic construct
  source 1..20: mol_type = other RNA
cagccccttattgttatacg

SEQ ID NO: 786 - RNA, 20 nt, synthetic construct
  source 1..20: mol_type = other RNA
tcgtataacaataaggggct

SEQ ID NO: 787 - RNA, 19 nt, synthetic construct
  source 1..19: mol_type = other RNA
cggtaatggacagagttat

SEQ ID NO: 788 - RNA, 19 nt, synthetic construct
  source 1..19: mol_type = other RNA
ataactctgtccattaccg

SEQ ID NO: 789 - DNA, 19 bp, synthetic construct
  source 1..19: mol_type = other DNA
tccgaacaagcaccgactg

SEQ ID NO: 790 - DNA, 19 bp, synthetic construct
  source 1..19: mol_type = other DNA
ggtccgactatgcgagtgt

SEQ ID NO: 791 - DNA, 21 bp, synthetic construct
  source 1..21: mol_type = other DNA
ggagcgagatccctccaaaat

SEQ ID NO: 792 - DNA, 23 bp, synthetic construct
  source 1..23: mol_type = other DNA
ggctgttgtcatacttctcatgg

SEQ ID NO: 793 - RNA, 20 nt, synthetic construct
  source 1..20: mol_type = other RNA
  modified_base 1..20: mod_base = OTHER; note = modified as descibed in table 9
cagccccttattgttatacg

SEQ ID NO: 794 - RNA, 20 nt, synthetic construct
  source 1..20: mol_type = other RNA
  modified_base 1..20: mod_base = OTHER; note = modified as descibed in table 9
tcgtataacaataaggggct

SEQ ID NO: 795 - RNA, 19 nt, synthetic construct
  source 1..19: mol_type = other RNA
  modified_base 1..19: mod_base = OTHER; note = modified as descibed in table 9
cggtaatggacagagttat

SEQ ID NO: 796 - RNA, 19 nt, synthetic construct
  source 1..19: mol_type = other RNA
  modified_base 1..19: mod_base = OTHER; note = modified as descibed in table 9
ataactctgtccattaccg